European Patent Specification EP 3 108 015 B1, published September 17, 2025. Title: Recombinant strain producing o-aminobenzoate and fermentative production of aniline from renewable resources via 2-aminobenzoic acid. Applicant: Bayer MaterialScience AG. The sequence listing filed with the application follows.

SEQUENCE LISTING (110 sequences)

SEQ ID NO: 1 - DNA, 1047 bp, Corynebacterium glutamicum
atgacttctccagcaacactgaaagttctcaacgcctacttggataaccccactccaaccctggaggaggcaattgaggtgttcaccccgctgaccgtgggtgaatacgatgacgtgcacatcgcagcgctgcttgccaccatccgtactcgcggtgagcagttcgctgatattgccggcgctgccaaggcgttcctcgcggcggctcgtccgttcccgattactggcgcaggtttgctagattccgctggtactggtggcgacggtgccaacaccatcaacatcaccaccggcgcatccctgatcgcagcatccggtggagtgaagctggttaagcacggcaaccgttcggtgagctccaagtccggctccgccgatgtgctggaagcgctgaatattcctttgggccttgatgtggatcgtgctgtgaagtggttcgaagcgtccaacttcaccttcctgttcgcacctgcgtacaaccctgcgattgcgcatgtgcagccggttcgccaggcgctgaaattccccaccatcttcaacacgcttggaccattgctgtccccggcgcgcccggagcgtcagatcatgggcgtggccaatgccaatcatggacagctcatcgccgaggtcttccgcgagttgggccgtacacgcgcgcttgttgtgcatggcgcaggcaccgatgagatcgcagtccacggcaccaccttggtgtgggagcttaaagaagacggcaccatcgagcattacaccatcgagcctgaggaccttggccttggccgctacacccttgaggatctcgtaggtggcctcggcactgagaacgccgaagctatgcgcgctactttcgcgggcaccggccctgatgcacaccgtgatgcgttggctgcgtccgcaggtgcgatgttctacctcaacggcgatgtcgactccttgaaagatggtgcacaaaaggcgctttccttgcttgccgacggcaccacccaggcatggttggccaagcacgaagagatcgattactcagaaaaggagtcttccaatgactag

SEQ ID NO: 2 - DNA, 69 bp, Artificial Sequence
  Artificial construct
atgacttctccagcaacactgtgtttaagtttagtggatcccggggaaaaggagtcttccaatgactag

SEQ ID NO: 3 - DNA, 32 bp, Artificial Sequence
  Artificial construct
gccctgcaggtaaaaaaaggatttgattcatg

SEQ ID NO: 4 - DNA, 32 bp, Artificial Sequence
  Artificial construct
gccctgcaggtaaaaaaaggatttgattcgtg

SEQ ID NO: 5 - DNA, 32 bp, Artificial Sequence
  Artificial construct
gccctgcaggtaaaaaaaggatttgattcttg

SEQ ID NO: 6 - DNA, 26 bp, Artificial Sequence
  Artificial construct
gccctgcaggtaaaaaaaggattatg

SEQ ID NO: 7 - DNA, 26 bp, Artificial Sequence
  Artificial construct
gccctgcaggtaaaaaaaggattgtg

SEQ ID NO: 8 - DNA, 26 bp, Artificial Sequence
  Artificial construct
gccctgcaggtaaaaaaaggattttg

SEQ ID NO: 9 - DNA, 312 bp, Corynebacterium glutamicum
gtgtgcatgactaatgcaggtgacaacttcgagatcaggatgccttctggcacggatgacccattgtccgatgcggagatccaaaagtatcgcgaggagatcaaccgcttggaccgcgaaatcctcgatgcggtgaaacgccgcacgaagatttcccaaaccatcggaaaaacacgcatgagctcgggcggaacacgtctcgtgcacacccgagaagtagcaatcatcaaccaattccgtgaagagatcggcgaggaaggccctgccctcgctggaattttgctgcgcatgggacgcggaaaactcggataa

SEQ ID NO: 10 - DNA, 60 bp, Artificial Sequence
  Artificial construct
atgactaatgcaggtgactgtttaagtttagtggatcccgggcgcggaaaactcggataa

SEQ ID NO: 11 - DNA, 32 bp, Artificial Sequence
  Artificial sequence
gccctgcaggacgtggcagaatagtgtgcatg

SEQ ID NO: 12 - DNA, 32 bp, Artificial Sequence
  Artificial sequence
gccctgcaggacgtggcagaatagtgtgcgtg

SEQ ID NO: 13 - DNA, 32 bp, Artificial Sequence
  Artificial sequence
gccctgcaggacgtggcagaatagtgtgcttg

SEQ ID NO: 14 - DNA, 27 bp, Artificial Sequence
  Artificial sequence
gccctgcaggacgtggcagaatagatg

SEQ ID NO: 15 - DNA, 27 bp, Artificial Sequence
  Artificial sequence
gccctgcaggacgtggcagaataggtg

SEQ ID NO: 16 - DNA, 27 bp, Artificial Sequence
  Artificial sequence
gccctgcaggacgtggcagaatagttg

SEQ ID NO: 17 - DNA, 270 bp, Corynebacterium glutamicum
atggcttccaagactgtaaccgtcggttcctccgttggcctgcacgcacgtccagcatccatcatcgctgaagcggctgctgagtacgacgacgaaatcttgctgaccctggttggctccgatgatgacgaagagaccgacgcgtcctcttccctcatgatcatggcgctgggcgcagagcacggcaacgaagttaccgtcacctccgacaacgctgaagctgttgagaagatcgctgcgcttatcgcacaggaccttgacgctgagtaa

SEQ ID NO: 18 - DNA, 63 bp, Artificial Sequence
  Artificial sequence
atggcttccaagactgtaacctgtttaagtttagtggatgggcaggaccttgacgctgagtaa

SEQ ID NO: 19 - DNA, 2052 bp, Corynebacterium glutamicum
atggcgtccaaactgacgacgacatcgcaacatattctggaaaaccttggtggaccagacaatattacttcgatgactcactgtgcgactcgccttcgcttccaagtgaaggatcaatccattgttgatcaacaagaaattgactccgacccatcagttcttggcgtagtaccccaaggatccaccggtatgcaggtggtgatgggtggatctgttgcaaactattaccaagaaatcctcaaacttgatggaatgaagcacttcgccgacggtgaagctacagagagttcatccaagaaggaatacggcggagtccgtggcaagtactcgtggattgactacgccttcgagttcttgtctgatactttccgaccaatcctgtgggccctgcttggtgcctcactgattattaccttgttggttcttgcggatactttcggtttgcaagacttccgcgctccaatggatgagcagcctgatacttatgtattcctgcactccatgtggcgctcggtcttctacttcctgccaattatggttggtgccaccgcagctcgaaagctcggcgcaaacgagtggattggtgcagctattccagccgcacttcttactccagaattcttggcactgggttctgccggcgataccgtcacagtctttggcctgccaatggttctgaatgactactccggacaggtattcccaccgctgattgcagcaattggtctgtactgggtggaaaagggactgaagaagatcatccctgaagcagtccaaatggtgttcgtcccattcttctccctgctgattatgatcccagcgaccgcattcctgcttggacctttcggcatcggtgttggtaacggaatttccaacctgcttgaagcgattaacaacttcagcccatttattctttccatcgttatcccattgctctacccattcttggttccacttggattgcactggccactaaacgccatcatgatccagaacatcaacaccctgggttacgacttcattcagggaccaatgggtgcctggaacttcgcctgcttcggcctggtcaccggcgtgttcttgctctccattaaggaacgaaacaaggccatgcgtcaggtttccctgggtggcatgttggctggtttgctcggcggcatttccgagccttccctctacggtgttctgctccgattcaagaagacctacttccgcctcctgccgggttgtttggcaggcggtatcgtgatgggcatcttcgacatcaaggcgtacgctttcgtgttcacctccttgcttaccatcccagcaatggacccatggttgggctacaccattggtatcgcagttgcattcttcgtttccatgttccttgttctcgcactggactaccgttccaacgaagagcgcgatgaggcacgtgcaaaggttgctgctgacaagcaggcagaagaagatctgaaggcagaagctaatgcaactcctgcagctccagtagctgctgcaggtgcgggagccggtgcaggtgcaggagccgctgctggcgctgcaaccgccgtggcagctaagccgaagctggccgctggggaagtagtggacattgtttccccactcgaaggcaaggcaattccactttctgaagtacctgacccaatctttgcagcaggcaagcttggaccaggcattgcaatccaaccaactggaaacaccgttgttgctccagcagacgctactgtcatccttgtccagaaatctggacacgcagtggcattgcgcttagatagcggagttgaaatccttgtccacgttggattggacaccgtgcaattgggcggcgaaggcttcaccgttcacgttgagcgcaggcagcaagtcaaggcgggggatccactgatcacttttgacgctgacttcattcgatccaaggatctacctttgatcaccccagttgtggtgtctaacgccgcgaaattcggtgaaattgaaggtattcctgcagatcaggcaaattcttccacgactgtgatcaaggtcaacggcaagaacgagtaa

SEQ ID NO: 20 - DNA, 63 bp, Artificial Sequence
  Artificial sequence
atggcgtccaaactgacgacgtgtttaagtttagtggatggggtcaacggcaagaacgagtaa

SEQ ID NO: 21 - DNA, 2760 bp, Corynebacterium glutamicum
atgactgattttttacgcgatgacatcaggttcctcggtcaaatcctcggtgaggtaattgcggaacaagaaggccaggaggtttatgaactggtcgaacaagcgcgcctgacttcttttgatatcgccaagggcaacgccgaaatggatagcctggttcaggttttcgacggcattactccagccaaggcaacaccgattgctcgcgcattttcccacttcgctctgctggctaacctggcggaagacctctacgatgaagagcttcgtgaacaggctctcgatgcaggcgacacccctccggacagcactcttgatgccacctggctgaaactcaatgagggcaatgttggcgcagaagctgtggccgatgtgctgcgcaatgctgaggtggcgccggttctgactgcgcacccaactgagactcgccgccgcactgtttttgatgcgcaaaagtggatcaccacccacatgcgtgaacgccacgctttgcagtctgcggagcctaccgctcgtacgcaaagcaagttggatgagatcgagaagaacatccgccgtcgcatcaccattttgtggcagaccgcgttgattcgtgtggcccgcccacgtatcgaggacgagatcgaagtagggctgcgctactacaagctgagccttttggaagagattccacgtatcaaccgtgatgtggctgttgagcttcgtgagcgtttcggcgagggtgttcctttgaagcccgtggtcaagccaggttcctggattggtggagaccacgacggtaacccttatgtcaccgcggaaacagttgagtattccactcaccgcgctgcggaaaccgtgctcaagtactatgcacgccagctgcattccctcgagcatgagctcagcctgtcggaccgcatgaataaggtcaccccgcagctgcttgcgctggcagatgcagggcacaacgacgtgccaagccgcgtggatgagccttatcgacgcgccgtccatggcgttcgcggacgtatcctcgcgacgacggccgagctgatcggcgaggacgccgttgagggcgtgtggttcaaggtctttactccatacgcatctccggaagaattcttaaacgatgcgttgaccattgatcattctctgcgtgaatccaaggacgttctcattgccgatgatcgtttgtctgtgctgatttctgccatcgagagctttggattcaacctttacgcactggatctgcgccaaaactccgaaagctacgaggacgtcctcaccgagcttttcgaacgcgcccaagtcaccgcaaactaccgcgagctgtctgaagcagagaagcttgaggtgctgctgaaggaactgcgcagccctcgtccgctgatcccgcacggttcagatgaatacagcgaggtcaccgaccgcgagctcggcatcttccgcaccgcgtcggaggctgttaagaaattcgggccacggatggtgcctcactgcatcatctccatggcatcatcggtcaccgatgtgctcgagccgatggtgttgctcaaggaattcggactcatcgcagccaacggcgacaacccacgcggcaccgtcgatgtcatcccactgttcgaaaccatcgaagatctccaggccggcgccggaatcctcgacgaactgtggaaaattgatctctaccgcaactacctcctgcagcgcgacaacgtccaggaagtcatgctcggttactccgattccaacaaggatggcggatatttctccgcaaactgggcgctttacgacgcggaactgcagctcgtcgaactatgccgatcagccggggtcaagcttcgcctgttccacggccgtggtggcaccgtcggccgcggtggcggaccttcctacgacgcgattcttgcccagcccaggggggctgtccaaggttccgtgcgcatcaccgagcagggcgagatcatctccgctaagtacggcaaccccgaaaccgcgcgccgaaacctcgaagccctggtctcagccacgcttgaggcatcgcttctcgacgtctccgaactcaccgatcaccaacgcgcgtacgacatcatgagtgagatctctgagctcagcttgaagaagtacgcctccttggtgcacgaggatcaaggcttcatcgattacttcacccagtccacgccgctgcaggagattggatccctcaacatcggatccaggccttcctcacgcaagcagacctcctcggtggaagatttgcgagccatcccatgggtgctcagctggtcacagtctcgtgtcatgctgccaggctggtttggtgtcggaaccgcattagagcagtggattggcgaaggggagcaggccacccaacgcattgccgagctgcaaacactcaatgagtcctggccatttttcacctcagtgttggataacatggctcaggtgatgtccaaggcagagctgcgtttggcaaagctctacgcagacctgatcccagatacggaagtagccgagcgagtctattccgtcatccgcgaggagtacttcctgaccaagaagatgttctgcgtaatcaccggctctgatgatctgcttgatgacaacccacttctcgcacgctctgtccagcgccgatacccctacctgcttccactcaacgtgatccaggtagagatgatgcgacgctaccgaaaaggcgaccaaagcgagcaagtgtcccgcaacattcagctgaccatgaacggtctttccactgcgctgcgcaactccggctag

SEQ ID NO: 22 - DNA, 63 bp, Artificial Sequence
  Artificial sequence
atgactgattttttacgcgattgtttaagtttagtggatggggcgctgcgcaactccggctag

SEQ ID NO: 23 - DNA, 1414 bp, Corynebacterium glutamicum
atgggcgtggatagacgaactaagattgtatgtaccctaggcccagcggtggctagtgcagatggaattctgcgtttggtagaagacggcatggatgttgctcgcctcaacttctcccatggtgaccacccagatcatgagcaaaactacaagtgggtccgcgaggcggcggagaagactggccgtgcagtcggtattctcgcagacctccaaggaccgaagatccgtcttggccgtttcactgacggcgcaaccgtgtgggaaaacggcgagaccattcggatcaccgttgacgatgtagagggaacgcacgatcgtgtgtccaccacctacaagaatctggcaaaagacgcgaagccaggcgaccgcctgctcgttgatgacggcaaggttggcctcgtctgcgtttccgtcgaaggtaacgacgtcatctgtgaggttgttgagggcggaccagtctccaacaacaagggtgtttccctgccaggtatggatatttccgtacctgcactgtccgaaaaggatatccgtgacctgcgcttcgccctgaagctcggcgtggactttattgcactgtccttcgtacgttccccagcagatgctgaactcgttcacaagatcatggacgaagaaggtcgtcgtgttcctgtgatcgccaagctggaaaagccagaggctgtcacctccctcgagccaatcgtgttggcattcgacgccgtcatggttgctcgtggtgacctcggcgttgaggttcctctggaggaggttccactggttcagaagcgcgcaatccagattgcccgtgagaacgcaaagccagttatcgtggcaacccagatgctggattccatgattgagaactcccgcccaacccgtgcggaagcttctgacgtggcaaacgctgtgctcgatggcgcagatgctgtcatgctttctggtgaaacttcagtgggcaaagatccgcacaacgttgtgcgcaccatgtctcgcattgttcgcttcgctgaaaccgacggtcgcgtcccagacctgacccacatccctcgcactaagcgtggcgttatttcctactctgcacgtgatatcgccgagcgcctcaacgctcgtgcattggttgcgttcaccacctctggtgataccgcaaagcgtgtggctcgtctgcacagccacctgccactgctcgtgttcactccaaatgaggcagttcgctctgagctggcgctgacctggggtgcaaccaccttcctgtgtccacctgtcagcgataccgatgacatgatgcgcgaagtcgaccgtgctcttttagcaatgcctgagtacaacaagggtgacatgatggttgttgttgcaggttcccctcctggtgttaccggtaacaccaacatgattcacgtccaccttcttggtgatctaa

SEQ ID NO: 24 - DNA, 63 bp, Artificial Sequence
  Artificial sequence
atgggcgtggatagacgaacttgtttaagtttagtggatgggacaaggattgcaaagctctaa

SEQ ID NO: 25 - DNA, 1860 bp, Corynebacterium glutamicum
atgaatgagtttgaccaggacattctccaggagatcaagactgaactcgacgagttaattctagaacttgatgaggtgacacaaactcacagcgaggccatcgggcaggtctccccaacccattacgttggtgcccgcaacctcatgcattacgcgcatcttcgcaccaaagacctccgtggcctgcagcaacgcctctcctctgtgggagctacccgcttgactaccaccgaaccagcagtgcaggcccgcctcaaggccgcccgcaatgttatcggagctttcgcaggtgaaggcccactttatccaccctcagatgtcgtcgatgccttcgaagatgccgatgagattctcgacgagcacgccgaaattctccttggcgaacccctaccggatactccatcctgcatcatggtcaccctgcccaccgaagccgccaccgacattgaacttgtccgtggcttcgccaaaagcggcatgaatctagctcgcatcaactgtgcacacgacgatgaaaccgtctggaagcagatgatcgacaacgtccacaccgttgcagaagaagttggccgggaaatccgcgtcagcatggacctcgccggaccaaaagtacgcaccggcgaaatcgccccaggcgcagaagtaggtcgcgcacgagtaacccgcgacgaaaccggaaaagtactgacgcccgcaaaactgtggatcaccgcccacggctccgaaccagtcccagcccccgaaagcctgcccggtcgccccgctctgccgattgaagtcaccccagaatggttcgacaaactagaaatcggcagcgtcatcaacgtcccagacacccgcggatcccgccgagcattcaccgtgaccagggtttttgatggcgcggtcctcgccgaaggcccacaaaaagcctacatctccaacggcaccctcctggaacacaactacgaccgctcccgggtctacggcatccccgccgtagttcagcgcatcaacctcaaagtcggcgaccgcctcatccttaccgacgaagaactcacctacgatccatccctcggatccggccgcacaccacgcatcagctgcacccttccacaagcagtcgatgcaattaaagtcgggcaccgcgtgcttttcgacgacggagccatcgccgcagtctgcatcgacaagacctccactgccgacggccacaacgacgtagaattggaagtcacccacgcccgcccacaaggcgtaaacctggccgcatacaagggaatcaacctcccagactccgaacttccactcccaagcctcactgaagaagacctccaacacctgcgctttgtcgtcaaatacgccgacatcgcagccatctccttcatccgaaacgtcgccgacgtggaatacctcctccaagcactcgccgacatcggagatccagtagccgtcgaacgccttggcctcgtccttaaaatcgagaccatcccaggctacgaaggcctcgcccaaatcctcctgaccggcatgcgccacgaaaacttcggcatcatgatcgcccgcggagacctcgccgtcgaactcggcttcgaccgcatggcagaagtcccccaactgatcatggcccttgccgaagccgcccacgtcccaaccatcttggccacccaagtcctggaaaacatggccaaaaacggactcccatctcgcgcagaaatcaccgacgcagcaatggcacttcgcgctgaatgcgtcatgctgaacaagggaccacacatcaacgacgccatcaaggtcctcaccgaaatgagccgcaaacttggtgcatcccaacgaaagagtaggctgctgctgcgcaaggtgaagagctgggaagagtaa

SEQ ID NO: 26 - DNA, 63 bp, Artificial Sequence
  Artificial sequence
atgaatgagtttgaccaggactgtttaagtttagtggatggggtgaagagctgggaagagtaa

SEQ ID NO: 27 - DNA, 1603 bp, Corynebacterium glutamicum
atggcggacatttcgaccacccaggtttggcaagacctgaccgatcattactcaaacttccaggcaaccactctgcgtgaacttttcaaggaagaaaaccgcgccgagaagtacaccttctccgcggctggcctccacgtcgacctgtcgaagaatctgcttgacgacgccaccctcaccaagctccttgcactgaccgaagaatctggccttcgcgaacgcattgacgcgatgtttgccggtgaacacctcaacaacaccgaagaccgcgctgtcctccacaccgcgctgcgccttcctgccgaagctgatctgtcagtagatggccaagatgttgctgctgatgtccacgaagttttgggacgcatgcgtgacttcgctactgcgctgcgctcaggcaactggttgggacacaccggccacacgatcaagaagatcgtcaacattggtatcggtggctctgacctcggaccagccatggctacgaaggctctgcgtgcatacgcgaccgctggtatctcagcagaattcgtctccaacgtcgacccagcagacctcgtttctgtgttggaagacctcgatgcagaatccacattgttcgtgatcgcttcgaaaactttcaccacccaggagacgctgtccaacgctcgtgcagctcgtgcttggctggtagagaagctcggtgaagaggctgtcgcgaagcacttcgtcgcagtgtccaccaatgctgaaaaggtcgcagagttcggtatcgacacggacaacatgttcggcttctgggactgggtcggaggtcgttactccgtggactccgcagttggtctttccctcatggcagtgatcggccctcgcgacttcatgcgtttcctcggtggattccacgcgatggatgaacacttccgcaccaccaagttcgaagagaacgttccaatcttgatggctctgctcggtgtctggtactccgatttctatggtgcagaaacccacgctgtcctaccttattccgaggatctcagccgttttgctgcttacctccagcagctgaccatggaatcaaatggcaagtcagtccaccgcgacggctcccctgtttccactggcactggcgaaatttactggggtgagcctggcacaaatggccagcacgctttcttccagctgatccaccagggcactcgccttgttccagctgatttcattggtttcgctcgtccaaagcaggatcttcctgccggtgagcgcaccatgcatgaccttttgatgagcaacttcttcgcacagaccaaggttttggctttcggtaagaacgctgaagagatcgctgcggaaggtgtcgcacctgagctggtcaaccacaaggtcatgccaggtaatcgcccaaccaccaccattttggcggaggaacttaccccttctattctcggtgcgttgatcgctttgtacgaacacatcgtgatggttcagggcgtgatttgggacatcaactccttcgaccaatggggtgttgaactgggcaaacagcaggcaaatgacctcgctccggctgtctctggtgaagaggatgttgactcgggagattcttccactgattcaaaataggtag

SEQ ID NO: 28 - DNA, 63 bp, Artificial Sequence
  Artificial sequence
atggcggacatttcgaccacctgtttaagtttagtggatgggtggtaccgcgcaaataggtag

SEQ ID NO: 29 - DNA, 975 bp, Corynebacterium glutamicum
atgagcaccgccgtagtttcacagaagaagtccacaacggcatccaaaattggacattggatgctcaataacggtgcgttggtggggctgattgcactgtgtgttggactttttattgcaacaccccactttctcaccattcctaacctgatcaacatcggtatccaatcggcgacggtggcgatcctggcgttcggcatgaccttcgtcatcgttaccgcaggcattgatttgtctgtgggatcagtggctgcgttgggtgcgatgacctcggcgtatttcttcgcggaagttggtttgccgggctggatcacgctgctgattggcctgttcatcggattgttggcgggtgcgatctctggcatttctattgcttatggcaagttgcctgcgtttattgccaccttggccatgatgtcgatcgccaggggaatcaccttggtcatttcccaaggctcaccaattcccagtgcaccagctgtgaacgctttggggcgcacctactttggcatcccgatgccgattctgatgatggcactggctggcattgtgtgttggtttattttgagccgcaccgtgctgggacggtccatgtacgccattggcggaaacatggaagcagcccgactatctggtctgccagtgaagaaaatcctggtcatggtctatgcactggctggtgtgtatgcagcacttgcgggtctggtcatgacgggacgcttgtcgtccgcgcagccgcaggcaggcgtgggatacgaactcgatgcgattgccgccgtggtcattggtggtgcgtcacttgctggcggaaccggaaaagcaacgggcactttgattggtgccatcttgttggccgtgatccgcaatggcttgaacattttgaacgtgtcctcgttctggcagcagattgtcatcggttgtgtcatcgcgcttgcggtgggcttcgatgtcatccgaaacaaaacctctaagtaa

SEQ ID NO: 30 - DNA, 1383 bp, Corynebacterium glutamicum
atgacaatgtgcgattacttcacaagctcaaggagaatttctgtggcttcccaaatttctggcggctggcaaagtgccaaacaccgcaccactgtttacatggtcctcgtagttgtgggcatttctattctttttgacggctacgatctagtgatctacggcgccgtgctgtcaacactacttgaagatccaacccagatcggtgcgctcagcccagcagtcgccggcacccttggttcctacgccatgatcggcgtgatgatcggtgctctatctgcaggtgccgttggtgaccgccttggtcgtcgcaaagttatgctcaccgcaatcgtctggttctctgtgggcatggcgctgaccgcgttcgcgtcctcgattgcgctgttcggtttcttgcgcttcctcaccggacttggcgtgggcatgatcgttgcaaccggcggcgcaatcatcgcggagttcgctccagcgaataggcgcaacttgttcaacgcaatcgtgtactccggtgtcccagccggtggcgtgctggcttctatccttgcactgctctttgaagatgtcatcggctggcgcggactcttcctcatcggtggttccccactactgttcctcctgccacttgcatacttcttcctcccagagtccccgcgctggctcacctcccgcggccgtgctgcggacgccaaagccctctgcgcacgctatgggctgccgacggaggaatttgtcgtcgaaaagcagcaggaaacaaagggcaccggattcgctggaattttctcctccaagtacctcatgggcaccattctcatcggcgcaatgagcttcatcgggctgctttcgacctacggcctgaacacctggttgccaaagatcatggaatccaacggcgcaacctcacatgattccctgtactccctgctgttcctcaacggcggcgcagtgttcggtggcctcatcgcatcctggttcgctgaccgcatcggcgcgaagaccgtgatcacctccaccttcgctctcgccgcgatctgcctcggagtcctgccaaacatctcctcctggccaatgatgtacaccgcaatcgcattcgcaggcgtcggcgtcctgggcacccaggttctcacctacggcctgacctcgaacttcttcggaaccgaatgccgcgcagcgggagttgcatggtgtgcaggattcggccgactcggcggaatcgtcggaccagcaatcggtggcctgatcatcggcgcaggattcggaccaagctccgcattcctcatcttcgcagcagctgccgcaatcggcgcggtctgcaccttgctgatcccgcgctccccagcagaagtagaggtcaaggtcgcgcaggaaccacttgcacgtgtctaa

SEQ ID NO: 31 - DNA, 1527 bp, Corynebacterium glutamicum
atgacggacatcaaggccacatcaagtacatcggccactacagcaccaacagcaggccgaccagcgcgtcgacttggacaaatttccctcgtcgcctgtctcggcggacttctcttcggctatgacaccggtgtcgccaacggcgccgaaggccacatggcacaagaactcggactcaacgtgctgcagctcggcgttgtcatcagttcactggttttcgctgcagcctttggcgcgctgttcgctgggcgtatctcggacgaaatcgggcgtcgaaaagcaattatcactttgtccgtgctgttcttcctcggatcaatcctcgtcgtattctcccccgccggtgagctggggcagttctacggaccaggatttgccaccttggtcaccgggcgcatcatgttgggtctcgcggttggcggcgcctccacagtagttccggtgtacctcgctgaactcgcaccactagaaatccgcggctccctgaccggccgaaacgagcttgctatcgtcaccggccagctgcttgccttcgtgatcaacgcgcttatcgccgtcaccctacacggagttattgatggaatctggcgcatcatgttcgccgtctgtgccctccctgccgtcgccctcttcctcggcatgctgcggatgccggaatcaccacgctggctggtcaaccaggggcgttacgacgacgcccgccgcgtcatggagaccgtccgtacccctgagcgtgcgaaagccgaaatggatgaaatcatcgcggtgcactctgaaaacaatgcggcacttcctggtgttaagcagtcttcgggccaggcttcaggccaggtttctagcaagcacacccacatgtccatcggcgaagtcctcagcaacaaatggctggttcgtctgctcatcgccggcatcggtgttgcagttgcccagcagctcaccggcatcaacgccatcatgtactacggaacccgcgtcctcgaggaatccggcatgagcgcagaaatggctgtggttgccaacattgctttcggtgccgttgccgtcatcggtggactgatcgcactgcgcaacatggaccgcctggatcgccgcaccaccttcatcatcggcctgtcactgaccaccaccttccaccttttgatcgcagctgccggcactctccttccagaaggtaactccattcgaccattcgccatcatgatccttgttgttgggttcgtgctctccatgcagactttcctcaacgttgcagtgtgggtgtggctggcggaaatcttcccagtccgaatgaagggtatcggcaccggtatttcggtattctgcggttggggcatcaatggcgtcctagcgttgttcttcccagcactggtctccggcgtgggtatcaccttctccttccttatcttcgcagtcgtcggagtcattgccctggcgttcgtcaccaagtttgttcctgaaacccgtggccgctcacttgaagaactcgatcacgcagcattcaccggccagattttcaagaaggcttaa

SEQ ID NO: 32 - DNA, 753 bp, Corynebacterium glutamicum
atgactgagactggatttggaattgatattggtggctccggcatcaaaggcgcccgcgttaaccttaagaccggtgagtttattgatgaacgcataaaaatcgccacccctaagccagcaaccccagaggctgtcgccgaagtagtcgcagagattatttctcaagccgaatgggagggtccggtcggaattaccctgccgtcggtcgttcgcgggcagatcgcgctatccgcagccaacattgacaagtcctggatcggcaccgatgtgcacgaactttttgaccgccacctaaatggccgagagatcaccgttctcaatgacgcagacgccgccggcatcgccgaagcaacctttggcaaccctgccgcacgcgaaggcgcagtcatcctgctgacccttggtacaggtattggttccgcattccttgtggatggccaactgttccccaacacagaactcggtcacatgatcgttgacggcgaggaagcagaacaccttgcagcagcatccgtcaaagaaaacgaggatctgtcatggaagaaatgggcgaagcacctgaacaaggtgctgagcgaatacgagaaacttttctccccatccgtcttcatcatcggtggcggaatttccagaaagcacgaaaagtggcttccattgatggagctagacactgacattgtcccagctgagctgcgcaatcgagccggaatcgtaggagctgctatggcagtaaaccaacacctcaccccataa

SEQ ID NO: 33 - DNA, 1083 bp, Corynebacterium glutamicum
atgaacatcccgtttgtccagcgcttcgatgaaggcctggaccctgttctagaagtactcggtggcaagggcgcttcactagtcaccatgacagatgctggaatgcccgttccacctggatttgtggtcactactgccagctttgatgagttcatccgtgaagcaggggttgctgaacacatcgataaattcctaaacgatctcgatgcagaagatgttaaggaagtggatcgagtttctgcgatcatccgcgatgagctgtgcagtcttgacgttccagagaatgctcgtttcgcagtgcaccaggcttatcgcgatctcatggaacgatgcggtggcgacgtcccggttgctgtccggtcatcggccactgccgaagacctgcccgatgcttccttcgcagggcaacaggacacctatctgtggcaagtcggtttgagcgctgtcactgaacacatccgtaaatgctgggcttcgctgttcacttcccgtgccattatctaccgtctgaaaaacaacatccccaatgagggcctctcgatggcggtagttgttcaaaaaatggtcaactctcgtgtcgcaggcgtggcaatcactatgaatccttccaacggcgaccgctcgaagatcaccatcgattcctcatggggtgttggtgaaatggtggtctcaggtgaagtgacaccagacaatatcttgctggacaagatcacgctgcaggttgtctccgaacacattggaagcaaacacgctgaactcatccccgatgccaccagtggaagcctcgtggaaaagcccgttgatgaagaacgcgcaaaccgccgcagtctgactgatgaggaaatgctcgctgtggcacaaatggctaagcgtgcagaaaaacactacaagtgcccacaagatatcgaatgggcgctggacgctgatctgccagatggagaaaaccttctgttattgcaatcccgcccggaaactatccactccaacggtgtgaagaaggaaaccccaactccgcaggctgccaaaaccataggcaccttcgatttcagctcaatcaccgtcgcaatgaccggcacgaagtaa

SEQ ID NO: 34 - DNA, 1743 bp, Corynebacterium glutamicum
atgttcaagccttttgaaactatcggtggtgagttcgctgtaaagtgcctcggccaatacaacgctcggcatttgatgatcccgaatgccaatggcatcgagttccgcgtgcatctgggatacctctatatgtcccctattccagtgcctgaagatcagattgcggaacgcgtccccatgttccaggaacgcatcacgcactacttccaaaactgggagccaatgctggcaaattggaaggagcgagtattaggaaccatcaatgagctggaatctctagagttcaagccactgcctgactacgtgcctatcgatgatattgtctccggaaaagccaaagacggcaccgaagtactcatggaaaacttcgatcggctcattcagctcgcctaccaaaactggcaataccactttgagttcctcaacttgggttacatcgcttacctagatttcttcaatttctgcaaggaagtcttcccagatatccctgatcaatcaatttcgatgatggttcagggcgtggatatggagctgttccgccccgatgatgaactaaagattctggcacagctagcggtcgaccttggcctgcaaactcactttgccaacccggatgatccgcaagctaccttggctgctatcgcaaaggcagaaggcggcgcgacatggatagcgcgctgggaagaagcacaagatccgtggttcaacttcaccgtcggtaatggcttctacggtcacgataaatactggatcgagcacctggaacttccactggggtacatcgcggattacatccgccgcctagatgaaggccaaaccatctcccgcccgaaagatgaactcatcgcagaaaaggaacgcgtggtggaagaataccgcgaccttttggatggagaacaactcgcgcagtttgatgctaaatgcggcctcgctgctactgcatacccctatgtggaaaaccataacttctacatcgagcactggaccatgtcagtattttggcgcaaagtacgcgaactttcccgcactctccagggctacggtttctgggagaacgaggatgacatgttgtacctcaaccgcactgaagtccgcgatgtcctcttcgacctggctactgcgtggggtgtcggcgcacccggtggtccaattggcacgatcatttggccggaagaaattgagcgaagaaaagcaattgtcaccgctttgaaaactgcccgaccagcgccagctcttaacactcctccagagtccatcaccgaacctttcacccgcatgctctggggaatcaccaccgaacaggtgcaatcatggttgggcaatgacgaggatgccgaagaaggaacccttaaaggcatggctgcatcccctggtgtggtggaaggctacgctcgagtaattctcagcgcagatgacctttcagaaatccagcaggatgaaatcctcgttgcccctgtaacagcaccttcttggggcccaatctttggcaaaatcaaggcaacagtcactgatattggtggcatgatgagccatgctgcgatcgtgtgccgcgaatacggcttgccggctgttactggaactggcgctgcatccaccaccatcaaaaccggcgattacctcaaggtcgatggaaccaagggcaaggttgtcattgttgatccagatgcgccacgcatcgaaggacccggcgcgcacagccatgcgcactcagtagcagcacatggggtggatacacatgcctag

SEQ ID NO: 35 - DNA, 24 bp, Artificial Sequence
  Artificial sequence
aaccaccgaaaggaggcccttcag

SEQ ID NO: 36 - DNA, 1833 bp, Corynebacterium glutamicum
atgactactgctgcaatcaggggccttcagggcgaggcgccgaccaagaataaggaactgctgaactggatcgcagacgccgtcgagctcttccagcctgaggctgttgtgttcgttgatggttcccaggctgagtgggatcgcatggcggaggatcttgttgaagccggtaccctcatcaagctcaacgaggaaaagcgtccgaacagctacctagctcgttccaacccatctgacgttgcgcgcgttgagtcccgcaccttcatctgctccgagaaggaagaagatgctggcccaaccaacaactgggctccaccacaggcaatgaaggacgaaatgtccaagcattacgctggttccatgaaggggcgcaccatgtacgtcgtgcctttctgcatgggtccaatcagcgatccggaccctaagctcggtgtgcagctcactgactccgagtacgttgtcatgtccatgcgcatcatgacccgcatgggtattgaagcgctggacaagatcggcgcgaacggcagcttcgtcaggtgcctccactccgttggtgctcctttggagccaggccaggaagacgttgcatggccttgcaacgacaccaagtacatcacccagttcccagagaccaaggaaatttggtcctacggttccggctacggcggaaacgcaatcctggcaaagaagtgctacgcactgcgtatcgcatctgtcatggctcgcgaagaaggatggatggctgagcacatgctcatcctgaagctgatcaacccagagggcaaggcgtaccacatcgcagcagcattcccatctgcttgtggcaagaccaacctcgccatgatcactccaaccatcccaggctggaccgctcaggttgttggcgacgacatcgcttggctgaagctgcgcgaggacggcctctacgcagttaacccagaaaatggtttcttcggtgttgctccaggcaccaactacgcatccaacccaatcgcgatgaagactatggaaccaggcaacaccctgttcaccaacgtggcactcaccgacgacggcgacatctggtgggaaggcatggacggcgacgccccagctcacctcattgactggatgggcaacgactggaccccagagtccgacgaaaacgctgctcaccctaactcccgttactgcgtagcaatcgaccagtccccagcagcagcacctgagttcaacgactgggaaggcgtcaagatcgacgcaatcctcttcggtggacgtcgcgcagacaccgtcccactggttacccagacctacgactgggagcacggcactatggttggtgcactgctcgcatccggtcagaccgcagcttccgcagaagcaaaggtcggcacactccgccacgacccaatggcaatgctcccattcattggctacaacgctggtgaatacctgcagaactggattgacatgggtaacaagggtggcgacaagatgccatccatcttcctggtcaactggttccgccgtggcgaagatggacgcttcctgtggcctggcttcggcgacaactctcgcgttctgaagtgggtcatcgaccgcatcgaaggccacgttggcgcagacgagaccgttgttggacacaccgctaaggccgaagacctcgacctcgacggcctcgacaccccaattgaggatgtcaaggaagcactgaccgctcctgcagagcagtgggcaaacgacgttgaagacaacgccgagtacctcactttcctcggaccacgtgttcctgcagaggttcacagccagttcgatgctctgaaggcccgcatttcagcagctcacgcttaa

SEQ ID NO: 37 - DNA, 1455 bp, Corynebacterium glutamicum
atggtgatcttcggtgtcactggcgacttggctcgaaagaagctgctccccgccatttatgatctagcaaaccgcggattgctgcccccaggattctcgttggtaggttacggccgccgcgaatggtccaaagaagactttgaaaaatacgtacgcgatgccgcaagtgctggtgctcgtacggagttccgtgaaaatgtttgggagcgcctcgccgagggtatggaatttgttcgcggcaactttgatgatgatgcagctttcgacaacctcgctgcaacactcaagcgcatcgacaaaacccgcggcaccgccggcaactgggcttactacctgtccattccaccagattccttcacagcggtctgccaccagctggagcgttccggcatggctgaatccaccgaagaagcatggcgccgcgtgatcatcgagaagcctttcggccacaacctcgaatccgcacacgagctcaaccagctggtcaacgcagtcttcccagaatcttctgtgttccgcatcgaccactatttgggcaaggaaacagttcaaaacatcctggctctgcgttttgctaaccagctgtttgagccactgtggaactccaactacgttgaccacgtccagatcacaatggctgaagatattggcttgggtggacgtgctggttactacgacggcatcggcgcagcccgcgacgtcatccagaaccacctgatccagctcttggctctggttgctatggaagaaccaatttctttcgtgccagcgcagctgcaggcagaaaagatcaaggtgctctctgcgacaaagccgtgctacccattggataaaacctccgctcgtggtcagtacgctgccggttggcagggctctgagttagtcaagggacttcgcgaagaagatggcttcaaccctgagtccaccactgagacttttgcggcttgtaccttagagatcacgtctcgtcgctgggctggtgtgccgttctacctgcgcaccggtaagcgtcttggtcgccgtgttactgagattgccgtggtgtttaaagacgcaccacaccagcctttcgacggcgacatgactgtatcccttggccaaaacgccatcgtgattcgcgtgcagcctgatgaaggtgtgctcatccgcttcggttccaaggttccaggttctgctatggaagtccgtgacgtcaacatggacttctcctactcagaatccttcactgaagaatcacctgaagcatacgagcgcctcattttggatgcgctgttagatgaatccagcctcttccctaccaacgaggaagtggaactgagctggaagattctggacccaattcttgaagcatgggatgccgatggagaaccagaggattacccagcgggtacgtggggtccaaagagcgctgatgaaatgctttcccgcaacggtcacacctggcgcaggccataa

SEQ ID NO: 38 - DNA, 960 bp, Corynebacterium glutamicum
atgatctttgaacttccggataccaccacccagcaaatttccaagaccctaactcgactgcgtgaatcgggcacccaggtcaccaccggccgagtgctcaccctcatcgtggtcactgactccgaaagcgatgtcgctgcagttaccgagtccaccaatgaagcctcgcgcgagcacccatctcgcgtgatcattttggtggttggcgataaaactgcagaaaacaaagttgacgcagaagtccgtatcggtggcgacgctggtgcttccgagatgatcatcatgcatctcaacggacctgtcgctgacaagctccagtatgtcgtcacaccactgttgcttcctgacacccccatcgttgcttggtggccaggtgaatcaccaaagaatccttcccaggacccaattggacgcatcgcacaacgacgcatcactgatgctttgtacgaccgtgatgacgcactagaagatcgtgttgagaactatcacccaggtgataccgacatgacgtgggcgcgccttacccagtggcggggacttgttgcctcctcattggatcacccaccacacagcgaaatcacttccgtgaggctgaccggtgcaagcggcagtacctcggtggatttggctgcaggctggttggcgcggaggctgaaagtgcctgtgatccgcgaggtgacagatgctcccaccgtgccaaccgatgagtttggtactccactgctggctatccagcgcctggagatcgttcgcaccaccggctcgatcatcatcaccatctatgacgctcatacccttcaggtagagatgccggaatccggcaatgccccatcgctggtggctattggtcgtcgaagtgagtccgactgcttgtctgaggagcttcgccacatggacccagatttgggctaccagcacgcactatccggcttgtccagcgtcaagctggaaaccgtctaa

SEQ ID NO: 39 - DNA, 14 bp, Artificial Sequence
  Artificial sequence
tttaggggcaaaaa

SEQ ID NO: 40 - DNA, 2031 bp, Corynebacterium glutamicum
atggacaccaaggctgtagacactgttcgtgtcctcgctgcagacgctgtagaaaactgtggctccggccacccaggcaccgcaatgagcctggctccccttgcatacaccttgtaccagcgggttatgaacgtagatccacaggacaccaactgggcaggccgtgaccgcttcgttctttcttgtggccactcctctttgacccagtacatccagctttacttgggtggattcggccttgagatggatgacctgaaggctctgcgcacctgggattccttgaccccaggacaccctgagtaccgccacaccaagggcgttgagatcaccactggccctcttggccagggtcttgcatctgcagttggtatggctatggctgctcgtcgtgagcgtggcctattcgacccaaccgctgctgagggcgaatccccattcgaccaccacatctacgtcattgcttctgatggtgaccttcaggaaggtgtcacctctgaggcatcctccatcgctggcacccagcagctgggcaacctcatcgtgttctgggatgacaaccgcatctccatcgaagacaacactgagatcgctttcaacgaggacgttgttgctcgttacaaggcttacggctggcagaccattgaggttgaggctggcgaggacgttgcagcaatcgaagctgcagtggctgaggctaagaaggacaccaagcgacctaccttcatccgcgttcgcaccatcatcggcttcccagctccaactatgatgaacaccggtgctgtgcacggtgctgctcttggcgcagctgaggttgcagcaaccaagactgagcttggattcgatcctgaggctcacttcgcgatcgacgatgaggttatcgctcacacccgctccctcgcagagcgcgctgcacagaagaaggctgcatggcaggtcaagttcgatgagtgggcagctgccaaccctgagaacaaggctctgttcgatcgcctgaactcccgtgagcttccagcgggctacgctgacgagctcccaacatgggatgcagatgagaagggcgtcgcaactcgtaaggcttccgaggctgcacttcaggcactgggcaagacccttcctgagctgtggggcggttccgctgacctcgcaggttccaacaacaccgtgatcaagggctccccttccttcggccctgagtccatctccaccgagacctggtctgctgagccttacggccgtaacctgcacttcggtatccgtgagcacgctatgggctccatcctcaacggcatttccctccacggtggcacccgcccatacggcggaaccttcctcatcttctccgactacatgcgtcctgcagttcgtcttgcagctctcatggagaccgacgcttactacgtctggacccacgactccatcggtctgggcgaagatggcccaacccaccagcctgttgaaaccttggctgcactgcgcgccatcccaggtctgtccgtcctgcgtcctgcagatgcgaacgagaccgcccaggcttgggctgcagcacttgagtacaaggaaggccctaagggtcttgcactgacccgccagaacgttcctgttctggaaggcaccaaggagaaggctgctgaaggcgttcgccgcggtggctacgtcctggttgagggttccaaggaaaccccagatgtgatcctcatgggctccggctccgaggttcagcttgcagttaacgctgcgaaggctctggaagctgagggcgttgcagctcgcgttgtttccgttccttgcatggattggttccaggagcaggacgcagagtacatcgagtccgttctgcctgcagctgtgaccgctcgtgtgtctgttgaagctggcatcgcaatgccttggtaccgcttcttgggcacccagggccgtgctgtctcccttgagcacttcggtgcttctgcggattaccagaccctgtttgagaagttcggcatcaccaccgatgcagtcgtggcagcggccaaggactccattaacggttaa

SEQ ID NO: 41 - DNA, 1992 bp, Corynebacterium glutamicum
atgtcctcacgtaaagagcttgccaatgctattcgtgcgctgagcatggacgcagtacagaaagccaaatccggtcacccgggtgcccctatgggtatggctgacattgccgaagtcctgtggcgtgatttcctgaaacacaacccgcagaatccgtcctgggctgaccgtgaccgcttcgtgctgtccaacggccacggctccatgctgatctacagcctgctgcacctcaccggttacgatctgccgatggaagaactgaaaaacttccgtcagctgcactctaaaactccgggtcacccggaagtgggttacaccgctggtgtggaaaccaccaccggtccgctgggtcagggtattgccaacgcagtcggtatggcgattgcagaaaaaacgctggcggcgcagtttaaccgtccgggccacgacattgtcgaccactacacctacgccttcatgggcgacggctgcatgatggaaggcatctcccacgaagtttgctctctggcgggtacgctgaagctgggtaaactgattgcattctacgatgacaacggtatttctatcgatggtcacgttgaaggctggttcaccgacgacaccgcaatgcgtttcgaagcatacggctggcacgttattcgcgacatcgacggtcatgacgcggcatctatcaaacgcgcagtagaagaagcgcgcgcagtgactgacaaaccttccctgctgatgtgcaaaaccatcatcggtttcggttccccgaacaaagccggtacccacgactcccacggtgcgccgctgggcgacgctgaaattgccctgacccgcgaacaactgggctggaaatatgcgccgttcgaaatcccgtctgaaatctatgctcagtgggatgcgaaagaagcaggccaggcgaaagaatccgcatggaacgagaaattcgctgcttacgcgaaagcatatccgcaggaagccgctgaatttacccgccgtatgaaaggcgaaatgccgtctgacttcgacgctaaagcgaaagagttcatcgctaaactgcaggctaatccggcgaaaatcgccagccgtaaagcgtctcagaatgctatcgaagcgttcggtccgctgttgccggagttcctcggcggttctgctgacctggcgccgtctaacctgaccctgtggtctggttctaaagcaatcaacgaagatgctgcgggtaactacatccactacggtgttcgcgagttcggtatgaccgcgattgctaacggtatctccctgcacggtggcttcctgccgtacacctccaccttcctgatgttcgtggaatacgcacgtaacgccgtacgtatggctgcgctgatgaaacagcgtcaggtgatggtttacacccacgactccatcggtctgggcgaagacggcccgactcaccagccggttgagcaggtcgcttctctgcgcgtaaccccgaacatgtctacatggcgtccgtgtgaccaggttgaatccgcggtcgcgtggaaatacggtgttgagcgtcaggacggcccgaccgcactgatcctctcccgtcagaacctggcgcagcaggaacgaactgaagagcaactggcaaacatcgcgcgcggtggttatgtgctgaaagactgcgccggtcagccggaactgattttcatcgctaccggttcagaagttgaactggctgttgctgcctacgaaaaactgactgccgaaggcgtgaaagcgcgcgtggtgtccatgccgtctaccgacgcatttgacaagcaggatgctgcttaccgtgaatccgtactgccgaaagcggttactgcacgcgttgctgtagaagcgggtattgctgactactggtacaagtatgttggcctgaacggtgctatcgtcggtatgaccaccttcggtgaatctgctccggcagagctgctgtttgaagagttcggcttcactgttgataacgttgttgcgaaagcaaaagaactgctgtaa

SEQ ID NO: 42 - DNA, 1083 bp, Corynebacterium glutamicum
atgtctcacattgatgatcttgcacagctcggcacttccacttggctcgacgacctctcccgcgagcgcattacttccggcaatctcagccaggttattgaggaaaagtctgtagtcggtgtcaccaccaacccagctattttcgcagcagcaatgtccaagggcgattcctacgacgctcagatcgcagagctcaaggccgctggcgcatctgttgaccaggctgtttacgccatgagcatcgacgacgttcgcaatgcttgtgatctgttcaccggcatcttcgagtcctccaacggctacgacggccgcgtgtccatcgaggttgacccacgtatctctgctgaccgcgacgcaaccctggctcaggccaaggagctgtgggcaaaggttgatcgtccaaacgtcatgatcaagatccctgcaaccccaggttctttgccagcaatcaccgacgctttggctgagggcatcagcgttaacgtcaccttgatcttctccgttgctcgctaccgcgaggtcatcgctgcgttcatcgagggcatcaagcaggctgctgcaaacggccacgacgtctccaagatccactctgtggcttccttcttcgtctcccgcgtcgacgttgagatcgacaagcgcctcgaggcaatcggctccgatgaggctttggctctgcgcggcaaggcaggcgttgccaacgctcagcgcgcttacgctgtgtacaaggagcttttcgacgccgccgagctgcctgaaggtgccaacactcagcgcccactgtgggcatccaccggcgtgaagaaccctgcgtacgctgcaactctttacgtttccgagctggctggtccaaacaccgtcaacaccatgccagaaggcaccatcgacgcggttctggagcagggcaacctgcacggtgacaccctgtccaactccgcggcagaagctgacgctgtgttctcccagcttgaggctctgggcgttgacttggcagatgtcttccaggtcctggagaccgagggtgtggacaagttcgttgcttcttggagcgaactgcttgagtctatggaagctcgcctgaagtag

SEQ ID NO: 43 - DNA, 951 bp, Corynebacterium glutamicum
atgaacgagttagacggcatcaaacagttcaccactgtcgtggcagacagcggcgatattgagtccattcgccattatcatccccaggatgccaccaccaatccttcgctgttactcaaagctgccggattatcacaatatgagcatttaatagacgatgctatcgcctggggtaaaaaaaatggcaagacccaggaacaacaggtggtcgcagcgtgtgacaaactggcggtcaatttcggtgctgaaatcctcaaaatcgtacccggtcgcgtgtcaacagaagttgatgcacgcctctcttttgataaagaaaagagtattgagaaggcgcgccatctggtggacttgtatcagcaacaaggcgttgagaaatcacgcattctgatcaagctggcttcgacctgggaaggtattcgcgcggcagaagagctggaaaaagaaggtattaactgcaacctgacgctgctgttttcttttgcacaggcacgggcctgtgcggaagcaggcgtttttctgatttcgccgtttgtcgggcgtatttatgactggtatcaggcacgcaagccgatggacccgtatgtggtggaagaagatccgggcgttaaatcggtgcgcaatatctacgactactataagcaacaccactatgaaaccattgtgatgggcgcgagcttccgtcgcaccgaacaaatcctcgccttaaccggctgcgatcgactgactatcgcaccgaatttactgaaggagctgcaggaaaaagtttcgccagtggtacgtaaattaatcccaccttctcagacgttcccacgcccagctcccatgagcgaagcggagttccgttgggagcacaatcaggatgcgatggcggtagaaaaactgtctgaaggcattcgtctgttcgccgttgatcaacgcaaactggaagaccttcttgccgccaaactataa

SEQ ID NO: 44 - DNA, 1452 bp, Corynebacterium glutamicum
atgtcttacacatcttttaaaggcgatgataaagccctcatcggcatagttttatcagttctcacattttggctttttgctcagtcaaccctaaatatcggcccagatatggcaactgatttagggatgagcgatggcaccatgaacatagctgtcgtggccgccgcgttattctgtggaacatttatcgtcgcagccggcggcatcgcagatgtctttggccgagtacgaatcatgatgattggcaacatccttaacatcctgggatctctcctcatcgccacggcaacgacttctttagccacccaaatggtgatcaccggccgagttctccaaggactggcagcagcggccatcatgtctgcatccctagcattagttaagacatattggttaggtactgaccgccaacgagcagtctccatttggtccattggttcatggggtggcaccggattctgcgcgcttttcgcgggtcttgttgtagcaagcccctttggttggagaggaatcttcgccctctgcgcgatcgtctccatcgttgctattgcccttacccgccacatcccggaatcccgtccggctcaatccattggcatgcatttggattggagtggcatcatcgttcttgccctcagtgttctatctcttgaattgtttattacccaaggtgaatcacttggctggacgcactggatgacctggactctccttgccgtttctttgacatttcttgcagttttcgtcttcattgaacgcatcgccagctggccagttctcgacttcaaccttttcaaagaccacgccttcagcggtgcgaccatcaccaacttcattatgagcgctactggcggagtagttgccgttgtcatgtgggttcagcaaatgggatggggtgtctccccaacaatctcgggactcaccagcatcggcttcgcagcctttgtcatccttttcattcgagttggagaaaaggccatgcagaaagttggcgcccgagcagtgatcatcaccgctggcatcttggtagcgaccgcgaccgccctcctaatgatcaccgcggtcagcgagtcaacgtacatcgtcatctccctcgccggcttctccctttatggccttggcctcggactcttcgccaccccagtcaccgatactgcgcttggaacacttcccaaagaccgtaccggcgctggtgcaggtgtattcaagatgtcctcttccctcggcgcagcactcggcatcgcaatctccacttcagtgttcctcgcacttcgcgacggcacctccatcaactccgacgtcgcactcgccggaacagtttcacttggcatcaacgttgtattcgcagcaacagccaccatcaccgcagcagtccttattccaaaagccgctggcaaagtctcacaaaccagcatcacccttcctgagccagctatcgctgtaaaaatctaa

SEQ ID NO: 45 - DNA, 174 bp, Artificial Sequence
  Artificial sequence
atggatctttcccttctcaaggaaaccctcggcaactacgagaccttcggtggcaacatcggtaccgctcttcagagcatcccaaccctgctcgattccatccttaacttcttcgacaacttcggagacctcgctgacaccaccggcgagaatctggataacttctcttcctaa

SEQ ID NO: 46 - DNA, 27 bp, Artificial Sequence
  Artificial sequence
gagaaatcctgaaaggaggcccttcag

SEQ ID NO: 47 - DNA, 138 bp, Artificial Sequence
  Artificial sequence
atggaaaacgtttacgagttccttggaaaccttgatgtcctttccggctccggcctcatcggctacgtcttcgacttcctcggcgcttccagcaagtgggctggcgcagttgctgacctcatcggtctgcttggctaa

SEQ ID NO: 48 - DNA, 1209 bp, Bacillus subtilis
atgaaaaatattattgcattgtcttctgtcccgcttgtgatgacactcgggaactccatgctgattcctgttcttccgatgatggagaaaaagctgtctgtgacttcatttcaagtatctttaatcattactgtatattcagtagtagcaattatttgcattccgattgccggatatttgtcggatcgtttcgggagaaaaaaaatattgcttccatgcctcctcattgcaggattggggggagccgtagctgcttttgcctcgacctatatgaaaaatccttatgctatgatcttggcggggcgggttcttcaaggcattggttctgcaggtgccgctccgattgtcatgccgtttatcggcgacctgtttaaaggagacgatgaaaaggtcagcgcgggtcttggcgatattgaaaccgccaacacgtcagggaaggtactgagtcccatacttggagccttactggcttcttggtattggtttgtaccgttttggtttattccgtttttctgtttgatcagctttttgctcgtattgtttttggtggccaagcctgaagaagatgaagatgcgcctgctgtttctgagtttattaagagtgtgaagaaaatttttaaacaggatggtcgctggctttatacggtcttcattatcgggtgtgtcattatgtttttgttatttggcgtattattttatttatcagatacgctggagaacaagtatgctattgacggagtagctaaaggcggattactggcaatcccacttttgtttttgtcaaccagttcttttatagctggcaaaaagatcggtaaagataaaggccgaatgaaattttgcgttgttacaggaatgattctgttaaccctttcgtttattgccttgtggtggaaccacagtttttattttttatttgtctttttaagctttggcgggattgggattggaatggctcttcctgctttagatgcattgataaccgaagggattgaaagtgaacaatgcggaaccatttcctccttttacaatagcatgcgctttataggagtagctctcggtccacctgtttttgctgcattaatgtctaatgcaaactggattattttcatactctcggcgttttgcagcatcgtttctttatttttagtgctctttactgtagatgctaaaaaaagtgaagaagaaaaaaacttagggacggtctag

SEQ ID NO: 49 - DNA, 1209 bp, Artificial Sequence
  ymfD BSU16825 codon optimized for Corynebacterium glutamicum
atgaagaacatcattgcgctgtcctctgtgccactcgttatgacccttggcaactctatgctgatccccgttctccccatgatggagaagaaactctcagtcacttcgtttcaggtgtccctcatcatcaccgtgtattctgtcgttgccatcatctgcattcccatcgctggctacctttcagatcgcttcggtcgcaagaagattctgctcccttgcttgctgatcgctggccttggcggagctgtcgcagcattcgcatctacgtacatgaagaacccgtatgctatgatccttgcgggtcgtgtccttcaaggcatcggctctgctggtgctgccccgattgtaatgccgttcattggtgacctctttaagggcgatgatgagaaagtatcagctggcctgggagatattgaaaccgccaatacgtccgggaaagtgcttagcccaattctcggagcccttttggctagctggtattggtttgtcccgttttggttcatccctttcttctgccttatttccttccttctggtgctctttctggtggccaaacctgaagaggacgaagatgccccagcagttagcgagttcatcaaatcggtcaagaaaatcttcaagcaggatggccgatggctgtacaccgtgttcatcatcgggtgtgtcattatgttccttctcttcggggtactgttttacctgagcgacaccctggaaaacaagtacgcaatcgacggtgttgcgaagggtggtttgctggcaattccactgctcttcctgtccacatcctcctttatcgctggtaagaaaatcggtaaagacaagggccgcatgaagttttgcgttgtgaccggaatgatcctgctcacattgtccttcatcgcactgtggtggaatcacagcttctacttcttgttcgtgttcctgtcttttggcggaatcggcattggcatggcgttgcctgcgttggatgccctcattaccgaagggatcgaatcggagcagtgtggaaccatttcctccttctacaactcaatgcggttcatcggagtcgctctgggtccaccagtctttgcagccctgatgtccaatgcgaactggatcatctttatcctgtcggcattctgctccattgtttccctgttcttggtgctgttcactgttgacgcaaagaagtccgaagaggagaagaacttgggcactgtttaa

SEQ ID NO: 50 - DNA, 2180 bp, Artificial Sequence
  Artificial sequence
atgagcacgaatccccatgttttctccctagatgtccgctatcacgaggatgcttctgcattgtttgcccacttgggtggcacaaccgcagatgatgcagccctgttggaattcgctgatatcaccaccaagaatggtatttcttccctcgcggtgttgaagagttcggtgcgcattacgtgcacgggcaacacggtggtaacgcagccgctgacggactcgggtagggcagtggttgcgcgcctaacgcagcagcttggccagtacaacaccgcagagaacacctttagcttccccgcctcagatgcggttgatgagcgcgagcgcctcaccgcaccaagcaccatcgaagtgctgcgcaagttgcagttcgagtccggctacagcgacgcgtccctgccactgctcatgggcggtttcgcgtttgatttcttagaaacctttgaaacgctccccgctgtcgaggagagcgtcaacacttaccccgattaccagttcgtcctcgcggaaatcgtcctggacatcaatcaccaggaccagaccgccaaactcgccggcgtctccaacgccccaggcgagctcgaggccgagctcaacaagctttcattgcttatcgacgccgccctccccgcaaccgaacacgcctaccaaaccacccctcacgacggcgacactcttcgcgttgtggctgatattcccgatgctcagttccgcacccagatcaatgagctgaaagaaaacatttacaacggtgacatctaccaagttgtcccggcgcgcactttcaccgcaccatgtcctgatgcattcgctgcttatctgcagctgcgtgccaccaacccgtcgccgtacatgttctatatccgtggcctcaacgaaggccgctcctatgaactttttggcgcatcccctgagtccaacctcaagttcaccgctgctaaccgtgagctgcagctgtacccaatcgcaggtacccgcccccgtggactcaacccagatggctccatcaacgatgagctagatatccgcaatgagttggatatgcgcactgatgccaaagagatcgcggagcacaccatgcttgtcgatctcgcccgcaacgacctggcccgcgtctcggtcccagcgtcgcgccgggttgcggatcttttgcaggtggatcgctattcccgcgtgatgcacttggtgtcccgtgtgacggcgacgttggacccagagcttgatgctttggacgcctatcgggcgtgcatgaatatgggcacgttgaccggcgctccgaagttgcgcgctatggagctgttgcgcggcgtcgaaaagcgcaggcgtggttcttatggtggggcagtggggtacctgcgcggcaatggcgatatggataattgcattgttattcgttcggcgtttgtccaggatggtgtggctgctgtgcaggctggtgctggtgtggtccgcgattctaatcctcaatctgaagccgatgagacgttgcacaaggcgtatgccgtgttgaatgccattgcgcttgctgctggttccactttggaggtcatccgatgacacacgttgttctcattgataatcacgattcttttgtctacaacctggtggatgcgttcgccgtggccggttataagtgcacggtgttccgcaatacggtgccagtggaaaccattttggcagccaacccggacctgatctgcctttcacctggacctggttaccctgccgatgcgggcaacatgatggcgctgatcgagcgcacactcggccagattcctttactgggtatttgcctcggctaccaggcactcatcgaataccacggcggcaaggttgagccttgtggccctgtgcacggcaccaccgacaacatgatccttactgatgcaggtgtgcagagccctgtttttgcaggtcttgccactgatgttgagcctgatcatccagaaatcccaggccgcaaggttccaattggccgttatcactcactgggctgcgtggttgccccagacggtattgaatcactaggtacctgttcctcggagattggtgatgtcatcatggcggcacgcaccaccgatggaaaggccattggcctgcagtttcaccctgagtcagtgctaagcccaacgggtcctgtcattttgtcccgctgtgtcgaacagcttctcgcgaactaa

SEQ ID NO: 51 - DNA, 2180 bp, Artificial Sequence
  Artificial sequence
atgagcacgaatccccatgttttctccctagatgtccgctatcacgaggatgcttctgcattgtttgcccacttgggtggcacaaccgcagatgatgcagccctgttggaacgcgctgatatcaccaccaagaatggtatttcttccctcgcggtgttgaagagttcggtgcgcattacgtgcacgggcaacacggtggtaacgcagccgctgacggactcgggtagggcagtggttgcgcgcctaacgcagcagcttggccagtacaacaccgcagagaacacctttagcttccccgcctcagatgcggttgatgagcgcgagcgcctcaccgcaccaagcaccatcgaagtgctgcgcaagttgcagttcgagtccggctacagcgacgcgtccctgccactgctcatgggcggtttcgcgtttgatttcttagaaacctttgaaacgctccccgctgtcgaggagagcgtcaacacttaccccgattaccagttcgtcctcgcggaaatcgtcctggacatcaatcaccaggaccagaccgccaaactcgccggcgtctccaacgccccaggcgagctcgaggccgagctcaacaagctttcattgcttatcgacgccgccctccccgcaaccgaacacgcctaccaaaccacccctcacgacggcgacactcttcgcgttgtggctgatattcccgatgctcagttccgcacccagatcaatgagctgaaagaaaacatttacaacggtgacatctaccaagttgtcccggcgcgcactttcaccgcaccatgtcctgatgcattcgctgcttatctgcagctgcgtgccaccaacccgtcgccgtacatgttctatatccgtggcctcaacgaaggccgctcctatgaactttttggcgcatcccctgagtccaacctcaagttcaccgctgctaaccgtgagctgcagctgtacccaatcgcaggtacccgcccccgtggactcaacccagatggctccatcaacgatgagctagatatccgcaatgagttggatatgcgcactgatgccaaagagatcgcggagcacaccatgcttgtcgatctcgcccgcaacgacctggcccgcgtctcggtcccagcgtcgcgccgggttgcggatcttttgcaggtggatcgctattcccgcgtgatgcacttggtgtcccgtgtgacggcgacgttggacccagagcttgatgctttggacgcctatcgggcgtgcatgaatatgggcacgttgaccggcgctccgaagttgcgcgctatggagctgttgcgcggcgtcgaaaagcgcaggcgtggttcttatggtggggcagtggggtacctgcgcggcaatggcgatatggataattgcattgttattcgttcggcgtttgtccaggatggtgtggctgctgtgcaggctggtgctggtgtggtccgcgattctaatcctcaatctgaagccgatgagacgttgcacaaggcgtatgccgtgttgaatgccattgcgcttgctgctggttccactttggaggtcatccgatgacacacgttgttctcattgataatcacgattcttttgtctacaacctggtggatgcgttcgccgtggccggttataagtgcacggtgttccgcaatacggtgccagtggaaaccattttggcagccaacccggacctgatctgcctttcacctggacctggttaccctgccgatgcgggcaacatgatggcgctgatcgagcgcacactcggccagattcctttactgggtatttgcctcggctaccaggcactcatcgaataccacggcggcaaggttgagccttgtggccctgtgcacggcaccaccgacaacatgatccttactgatgcaggtgtgcagagccctgtttttgcaggtcttgccactgatgttgagcctgatcatccagaaatcccaggccgcaaggttccaattggccgttatcactcactgggctgcgtggttgccccagacggtattgaatcactaggtacctgttcctcggagattggtgatgtcatcatggcggcacgcaccaccgatggaaaggccattggcctgcagtttcaccctgagtcagtgctaagcccaacgggtcctgtcattttgtcccgctgtgtcgaacagcttctcgcgaactaa

SEQ ID NO: 52 - DNA, 2177 bp, Artificial Sequence
  Artificial sequence
atgcaaacacaaaaaccgactctcgaactgctaacctgcgaaggcgcttatcgcgacaatcccaccgcgctttttcaccagttgtgtggggatcgtccggcaacgctgctgctggaattcgcagatatcgacagcaaagatgatttaaaaagcctgctgctggtagacagtgcgctgcgcattacagctttaggtgacactgtcacaatccaggcactttccggcaacggcgaagccctcctggcactactggataacgccctgcctgcgggtgtggaaagtgaacaatcaccaaactgccgtgtgctgcgcttcccccctgtcagtccactgctggatgaagacgcccgcttatgctccctttcggtttttgacgctttccgtttattgcagaatctgttgaatgtaccgaaggaagaacgagaagccatgttcttcggcggcctgttctcttatgaccttgtggcgggatttgaagatttaccgcaactgtcagcggaaaataactgccctgatttctgtttttatctcgctgaaacgctgatggtgattgaccatcagaaaaaaagcacccgtattcaggccagcctgtttgctccgaatgaagaagaaaaacaacgtctcactgctcgcctgaacgaactacgtcagcaactgaccgaagccgcgccgccgctgccagtggtttccgtgccgcacatgcgttgtgaatgtaatcagagcgatgaagagttcggtggcgtagtgcgtttgttgcaaaaagcgattcgcgctggagaaattttccaggtggtgccatctcgccgtttctctctgccctgcccgtcaccgctggcggcctattacgtgctgaaaaagagtaatcccagcccgtacatgttttttatgcaggataatgatttcaccctatttggcgcgtcgccggaaagctcgctcaagtatgatgccaccagccgccagattgaaatctacccgattgccggaacacgcccacgcggtcgtcgcgccgatggttcactggacagggatctcgacagccgtattgaactggaaatgcgtaccgatcataaagagctgtctgaacatctgatgctggttgatctcgcccgtaatgatctggcacgcatttgcacccccggcagccgctacgtcgccgatctcaccaaagttgaccgttattcctatgtgatgcacctcgtctctcgcgtagtcggcgaactgcgtcacgatcttgacgccctgcacgcttatcgcgcctgtatgaatatggggacgttaagcggtgcgccgaaagtacgcgctatgcagttaattgccgaggcggaaggtcgtcgccgcggcagctacggcggcgcggtaggttatttcaccgcgcatggcgatctcgacacctgcattgtgatccgctcggcgctggtggaaaacggtatcgccaccgtgcaagcgggtgctggtgtagtccttgattctgttccgcagtcggaagccgacgaaacccgtaacaaagcccgcgctgtactgcgcgctattgccaccgcgcatcatgcacaggagactttctgatggctgacattctgctgctcgataatatcgactcttttacgtacaacctggcagatcagttgcgcagcaatgggcataacgtggtgatttaccgcaaccatattccggcgcaaaccttaattgaacgcctggcgaccatgagcaatccggtgctgatgctttctcctggccccggtgtgccgagcgaagccggttgtatgccggaactcctcacccgcttgcgtggcaagctgcccattattggcatttgcctcggacatcaggcgattgtcgaagcttacgggggctatgtcggtcaggcgggcgaaattctccacggtaaagcctccagcattgaacatgacggtcaggcgatgtttgccggattaacaaacccgctgccggtggcgcgttatcactcgctggttggcagtaacattccggccggtttaaccatcaacgcccattttaatggcatggtgatggcagtacgtcacgatgcggatcgcgtttgtggattccagttccatccggaatccattctcaccacccagggcgctcgcctgctggaacaaacgctggcctgggcgcagcagaaactagagccagccaacacgctgcaaccgattctgtaa

SEQ ID NO: 53 - DNA, 2177 bp, Artificial Sequence; identical to SEQ ID NO: 52
  Artificial sequence

SEQ ID NO: 54 - DNA, 2177 bp, Artificial Sequence
  Artificial sequence
atgcaaacacaaaaaccgactctcgaactgctaacctgcgaaggcgcttatcgcgacaatcccaccgcgctttttcaccagttgtgtggggatcgtccggcaacgctgctgctggaatccgcagatatcgacagcaaagatgatttaaaaagcctgctgctggtagacagtgcgctgcgcattacagctttaggtgacactgtcacaatccaggcactttccggcaacggcgaagccctcctggcactactggataacgccctgcctgcgggtgtggaaagtgaacaatcaccaaactgccgtgtgctgcgcttcccccctgtcagtccactgctggatgaagacgcccgcttatgctccctttcggtttttgacgctttccgtttattgcagaatctgttgaatgtaccgaaggaagaacgagaagccatgttcttcggcggcctgttctcttatgaccttgtggcgggatttgaagatttaccgcaactgtcagcggaaaataactgccctgatttctgtttttatctcgctgaaacgctgatggtgattgaccatcagaaaaaaagcacccgtattcaggccagcctgtttgctccgaatgaagaagaaaaacaacgtctcactgctcgcctgaacgaactacgtcagcaactgaccgaagccgcgccgccgctgccagtggtttccgtgccgcacatgcgttgtgaatgtaatcagagcgatgaagagttcggtggcgtagtgcgtttgttgcaaaaagcgattcgcgctggagaaattttccaggtggtgccatctcgccgtttctctctgccctgcccgtcaccgctggcggcctattacgtgctgaaaaagagtaatcccagcccgtacatgttttttacgcaggataatgatttcaccctatttggcgcgtcgccggaaagctcgctcaagtatgatgccaccagccgccagattgaaatctacccgattgccggaacacgcccacgcggtcgtcgcgccgatggttcactggacagggatctcgacagccgtattgaactggaaatgcgtaccgatcataaagagctgtctgaacatctgatgctggttgatctcgcccgtaatgatctggcacgcatttgcacccccggcagccgctacgtcgccgatctcaccaaagttgaccgttattcctatgtgatgcacctcgtctctcgcgtagtcggcgaactgcgtcacgatcttgacgccctgcacgcttatcgcgcctgtatgaatatggggacgttaagcggtgcgccgaaagtacgcgctatgcagttaattgccgaggcggaaggtcgtcgccgcggcagctacggcggcgcggtaggttatttcaccgcgcatggcgatctcgacacctgcattgtgatccgctcggcgctggtggaaaacggtatcgccaccgtgcaagcgggtgctggtgtagtccttgattctgttccgcagtcggaagccgacgaaacccgtaacaaagcccgcgctgtactgcgcgctattgccaccgcgcatcatgcacaggagactttctgatggctgacattctgctgctcgataatatcgactcttttacgtacaacctggcagatcagttgcgcagcaatgggcataacgtggtgatttaccgcaaccatattccggcgcaaaccttaattgaacgcctggcgaccatgagcaatccggtgctgatgctttctcctggccccggtgtgccgagcgaagccggttgtatgccggaactcctcacccgcttgcgtggcaagctgcccattattggcatttgcctcggacatcaggcgattgtcgaagcttacgggggctatgtcggtcaggcgggcgaaattctccacggtaaagcctccagcattgaacatgacggtcaggcgatgtttgccggattaacaaacccgctgccggtggcgcgttatcactcgctggttggcagtaacattccggccggtttaaccatcaacgcccattttaatggcatggtgatggcagtacgtcacgatgcggatcgcgtttgtggattccagttccatccggaatccattctcaccacccagggcgctcgcctgctggaacaaacgctggcctgggcgcagcagaaactagagccagccaacacgctgcaaccgattctgtaa

SEQ ID NO: 55 - DNA, 1053 bp, Artificial Sequence
  Artificial sequence
atgaattatcagaacgacgatttacgcatcaaagaaatcaaagagttacttcctcctgtcgcattgctggaaaaattccccgctactgaaaatgccgcgaatacggttgcccatgcccgaaaagcgatccataagatcctgaaaggtaatgatgatcgcctgttggttgtgattggcccatgctcaattcatgatcctgtcgcggcaaaagagtatgccactcgcttgctggcgctgcgtgaagagctgaaagatgagctggaaatcgtaatgcgcgtctattttgaaaagccgcgtaccacggtgggctggaaagggctgattaacgatccgcacatggataatagcttccagatcaacgacggtctgcgtatagcccgtaaattgctgcttgatattaacgacagcggtctgccagcggcaggtgagtttctcaatatgatcaccccacaatatctcgctgacctgatgagctggggcgcaattggcgcacgtaccaccgaatcgcaggtgcaccgcgaactggcatcagggctttcttgtccggtcggcttcaaaaatggcaccgacggtacgattaaagtggctatcgatgccattaatgccgccggtgcgccgcactgcttcctgtccgtaacgaaatgggggcattcggcgattgtgaataccagcggtaacggcgattgccatatcattctgcgcggcggtaaagagcctaactacagcgcgaagcacgttgctgaagtgaaagaagggctgaacaaagcaggcctgccagcacaggtgatgatcgatttcagccatgctaactcgtccaaacaattcaaaaagcagatggatgtttgtgctgacgtttgccagcagattgccggtggcgaaaaggccattattggcgtgatggtggaaagccatctggtggaaggcaatcagagcctcgagagcggggagccgctggcctacggtaagagcatcaccgatgcctgcatcggctgggaagataccgatgctctgttacgtcaactggcgaatgcagtaaaagcgcgtcgcgggtaa

SEQ ID NO: 56 - DNA, 1101 bp, Artificial Sequence
  Artificial sequence
atgagttctccagtctcactcgaaaacgcggcgtcaaccagcaacaagcgcgtcgtggctttccacgagctgcctagccctacagacctcatcgccgcaaacccactgacaccaaagcaggcttccaaggtggagcaggatcgccaggacatcgctgatatcttcgctggcgacgatgaccgcctcgttgtcgttgtgggaccttgctcagttcacgatcctgaagcagccatcgattacgcaaaccgcctggctccgctggcaaagcgccttgatcaggacctcaagattgtcatgcgcgtgtacttcgagaagcctcgcaccatcgtcggatggaagggattgatcaatgatcctcacctcaacgaaacctacgacatcccagagggcttgcgcattgcgcgcaaagtgcttatcgacgttgtgaaccttgatctcccagtcggctgcgaattcctcgaaccaaacagccctcagtactacgccgacactgtcgcatggggagcaatcggcgctcgtaccaccgaatctcaggtgcaccgccagctggcttctgggatgtgtatgccaattggtttcaagaacggaactgacggaaacatccaggttgcagtcgacgcggtacaggctgcccagaacccacacttcttcttcggaacctccgacgacggcgcgctgagcgtcgtggagaccgcaggcaacagcaactcccacatcattttgcgcggcggtacctccggcccgaatcatgatgcagcttcggtggaggccgtcgtcgagaagcttggtgaaaacgctcgtctcatgatcgatgcttcccatgctaactccggcaaggatcatatccgacaggttgaggttgttcgtgaaatcgcagagcagatttctggcggttctgaagctgtggctggaatcatgattgagtccttcctcgttggtggcgcacagaaccttgatcctgcgaaattgcgcatcaatggcggtgaaggcctggtgtacggacagtctgtgaccgataagtgcatcgatattgacaccaccatcgatttgctcgctgagctggccgcagcagtaagggaacgccgagcagcagccaagtaa

SEQ ID NO: 57 - DNA, 1089 bp, Corynebacterium glutamicum
atggagaggattgtcgttactctcggggaacgtagttacccaattaccatcgcatctggtttgtttaatgaaccagcttcattcttaccgctgaaatcgggcgagcaggtcatgttggtcaccaacgaaaccctggctcctctgtatctcgataaggtccgcggcgtacttgaacaggcgggtgttaacgtcgatagcgttatcctccctgacggcgagcagtataaaagcctggctgtactcgataccgtctttacggcgttgttacaaaaaccgcatggtcgcgatactacgctggtggcgcttggcggcggcgtagtgggcgatctgaccggcttcgcggcggcgagttatcagcgcggtgtccgtttcattcaagtcccgacgacgttactgtcgcaggtcgattcctccgttggcggcaaaactgcggtcaaccatcccctcggtaaaaacatgattggcgcgttctaccaacctgcttcagtggtggtggatctcgactgtctgaaaacgcttcccccgcgtgagttagcgtcggggctggcagaagtcatcaaatacggcattattcttgacggtgcgttttttaactggctggaagagaatctggatgcgttgttgcgtctggacggtccggcaatggcgtactgtattcgccgttgttgtgaactgaaggcagaagttgtcgccgccgacgagcgcgaaaccgggttacgtgctttactgaatctgggacacacctttggtcatgccattgaagctgaaatggggtatggcaattggttacatggtgaagcggtcgctgcgggtatggtgatggcggcgcggacgtcggaacgtctcgggcagtttagttctgccgaaacgcagcgtattataaccctgctcaagcgggctgggttaccggtcaatgggccgcgcgaaatgtccgcgcaggcgtatttaccgcacatgctgcgtgacaagaaagtccttgcgggagagatgcgcttaattcttccgttggcaattggtaagagtgaagttcgcagcggcgtttcgcacgagcttgttcttaacgccattgccgattgtcaatcagcgtaa

SEQ ID NO: 58 - DNA, 1098 bp, Artificial Sequence
  Artificial sequence
atgagcgcagtgcagattttcaacaccgtccacgtcaatggatcttccccctatgatgtccacattggttccggcctcaacgagctcattgttcagcgcgcagcggaatcaggcgcggagcaggtagcgattttgcaccagcccagcatggatgacattgcatccgagttggatgcagcactagtcgctgctggtttgaaggtcctgcaccttaatgttcccgatgcggaaaacggcaagtccttggaagtagcggggcagtgctgggatgaattgggtggcgcagcattcggccgccgcgatatcgtcatcggacttggtggcggtgctgccacagacctcgcgggattcgtcgctgctgcatggatgcgtggcgtgcgcgtcattcaggttccaaccaccttgttggctatggtggacgctgcggtgggcggcaagactggcatcaataccgccgcaggcaagaaccttgtgggcgcgttccacgagcctgacgcagtattcattgacaccgatcgcctagccaccctgcctgacgcggaaatcatcgcgggttccgccgaaatcatcaaaactggtttcatcgccgacccagaaatcctgcgcctttacgaaactgatcccgcagcctgcctgaagaaagaagtcgaaggctcccacctacctgaactgatttggcgctccgtcaccgtcaagggctccgtggtcggccaagacctcaaagaatctagcctgcgcgaaatcctcaactacggacacacctttgcccacgccgtcgaactccgcgaaaacttccgctggcgccacggcaatgccgttgcagtgggcatgatgttcatcgccaacctctcccacaagctcgggcttatcgacgcgcccctcctcgagcgccaccgctcaatcctggcggccatcggtctgcccacttcctacgaaggcggagccttcgacgagctttacgacggtatgacccgcgacaagaaaaaccgcgacggcaacatccgcttcgtcgcactgaccgccgtgggcgaggttacccgcattgaggggccctcaaaacaagatttacagagtgcttatgaggcaatcagccactaa

SEQ ID NO: 59 - DNA, 525 bp, Corynebacterium glutamicum
atgacacaacctctttttctgatcgggcctcggggctgtggtaaaacaacggtcggaatggcccttgccgattcgcttaaccgtcggtttgtcgataccgatcagtggttgcaatcacagctcaatatgacggtcgcggagatcgtcgaaagggaagagtgggcgggatttcgcgccagagaaacggcggcgctggaagcggtaactgcgccatccaccgttatcgctacaggcggcggcattattctgacggaatttaatcgtcacttcatgcaaaataacgggatcgtggtttatttgtgtgcgccagtatcagtcctggttaaccgactgcaagctgcaccggaagaagatttacggccaaccttaacgggaaaaccgctgagcgaagaagttcaggaagtgctggaagaacgcgatgcgctatatcgcgaagttgcgcatattatcatcgacgcaacaaacgaacccagccaggtgatttctgaaattcgcagcgccctggcacagacgatcaattgttga

SEQ ID NO: 60 - DNA, 573 bp, Corynebacterium glutamicum
atggagcgtaatgaagtgaatgatcaaattcacttagatcatcaatcagatgacacctctgaatgctcctgcccgatcgtggttcttgtgggtttgccaggagctggaaaatccaccattggacgtcgattagcgcgcgccttaaacactgaactcgtcgactccgacgaactgattgagcgcgccaccggaaaagcctgtggcgccgtgttcagcgagctcggcgagccagccttccgcgagctcgaggccatccacgtggccgaagcactgaaatcctccggagtggtgagcttgggaggcggatctgtgctgacagaatccacccgtgaactgctcaaaggccaggacgtggtctggatcgacgtgccagtagaagaaggcatcaggcgcaccgcaaacgagcgttcccgccccgtgctgcaagccgccgaccccgccgagcactaccgcaacctggtgaaagtgcgcaccccgttgtacgaagaggtggcaacctaccgacttcgcaccaacaaccgcagcccccagcaagtggtggcagcagtgttgcatcatctagaaatcgattaa

SEQ ID NO: 61 - DNA, 1434 bp, Artificial Sequence
  Artificial sequence
gtggcgtttgaaaccccggaagaaattgtcaagttcatcaaggatgaaaacgtcgagttcgttgacgttcgattcaccgaccttcccggcaccgagcagcacttcagcatcccagctgccagcttcgatgcagatacaatcgaagaaggtctcgcattcgacggctcctcgatccgtggcttcaccacgatcgacgaatctgacatgaatctcctgccagacctcggaacggccacccttgatccattccgcaaggcaaagaccctgaacgttaagttcttcgttcacgatcctttcacccgcgaggcattctcccgcgacccacgcaacgtggcacgcaaggcagagcagtacctggcatccaccggcattgcagacacctgcaacttcggcgccgaggctgagttctacctcttcgactccgttcgctactccaccgagatgaactccggcttctacgaagtagataccgaagaaggctggtggaaccgtggcaaggaaaccaacctcgacggcaccccaaacctgggcgcaaagaaccgcgtcaagggtggctacttcccagtagcaccatacgaccaaaccgttgacgtgcgcgatgacatggttcgcaacctcgcagcttccggcttcgctcttgagcgtttccaccacgaagtcggtggcggacagcaggaaatcaactaccgcttcaacaccatgctccacgcggcagatgatatccagaccttcaagtacatcatcaagaacaccgctcgcctccacggcaaggctgcaaccttcatgcctaagccactggctggcgacaacggttccggcatgcacgctcaccagtccctctggaaggacggcaagccactcttccacgatgagtccggctacgcaggcctgtccgacatcgcccgctactacatcggcggcatcctgcaccacgcaggcgctgttctggcgttcaccaacgcaaccctgaactcctaccaccgtctggttccaggcttcgaggctccaatcaacctggtgtactcacagcgcaaccgttccgctgctgtccgtatcccaatcaccggatcaaacccgaaggcaaagcgcatcgaattccgcgctccagacccatcaggcaacccatacctgggctttgcagcgatgatgatggccggcctcgacggcatcaagaaccgcatcgagccacacgctccagtggacaaggacctctacgaactaccaccagaggaagctgcatccattccacaggcaccaacctccctggaagcatccctgaaggcactgcaggaagacaccgacttcctcaccgagtctgacgtcttcaccgaggatctcatcgaggcgtacatccagtacaagtacgacaacgaaatctccccagttcgcctgcgcccaaccccgcaggaattcgaattgtacttcgactgctaa

SEQ ID NO: 62 - DNA, 1341 bp, Artificial Sequence
  Artificial sequence
atgaacagcgaacaggaatttgtactcagcgccattgaagaacgcgacattaagtttgtgcgtctatggttcactgacattcttggccacttgaagtcagtggttgtggctcctgcagaactagagtctgcgttggaagaaggcatcggattcgatggctcagccattgagggctacgcgcgtatctcggaagcggacaccattgcccgcccagatccatcgacattccaggtcctcccactagaagcgggcatctcaaaactgcaggcagcacgcctgttttgcgatgtcacgatgccagacggacagccatctttttctgacccgcgccaagtgctgcgcaggcaggtccaactagctgcagatgaaggcttgacctgcatgatctcaccagagattgagttctatttggtgcaaagccttcgcaccaacggactgccacctgtgcccactgacaacggcggatatttcgaccaagccacattcaatgaggcgccgaatttccgtcgaaacgcgatggtagcgctggaggaactcggcatccctgtcgagttctcccaccatgaaactgcacctggccagcaagaaatcgatttacgccatgcggatgcgctcactatggccgacaacatcatgaccttccgctacatcatgaaacaggtggcaagggaccaaggcgtcggggcatcatttatgcccaagccattccaagaacatgcaggctccgccatgcacacgcacatgtccttatttgagggcgataccaacgcgttccacgatccagacgattcttacatgctgtccaaaaccgcaaaacagttcatcgctggaatcttgcatcacgctccagaattcaccgctgtgaccaaccagtgggtcaattcctacaaacgcatcgtgtacggaaacgaagctccaactgcggcaacctggggtgtatctaatcgttctgcgctggttcgtgttcctacctaccgtttgaataaggaggagtcgcgccgggtggaggtgcgtcttcctgataccgcttgtaacccatatttggcgttttcagtgatgctcggcgctggtttgaaaggcattaaagaaggttatgagctcgacgagccagctgaggacgatatctccaacttgagcttccgggaacgtcgcgctatgggctacaacgatctgccaagcagccttgatcaggcactgcgccaaatggaaaagtcagagcttgttgctgacatcctcggtgagcacgtttttgagtttttcttgcgcaataagtggcgtgaatggcgtgactaccaagagcagatcactccgtgggagctccgaaacaatcttgattactag

SEQ ID NO: 63 - DNA, 1880 bp, Corynebacterium glutamicum
atggatatcaagagtgcgttgagccgtatcgtcgggcagttggacctgactaccgaagaaatgcgcgaggtcatgcgccagatcatgaccggtcagtgcagcgaggcgcagataggcgctttcctgatgggcatgcgcatgaaaagcgaaagcatcgacgaaatcgtcggtgcggtgtcggtgatgcgtgagctggccgaaaaggtcgagctgcaaagcctcgatggtgtcgtcgatattgtcgggaccggtggtgatggcgccaacatcttcaacgtgtccaccgcttcgtccttcgtcctggcggcggcgggttgcccggtggccaagcatggtaaccgcgcagtctcgggcaagagcggcagtgccgacctgctggaagctgccggcatctacctgaacctgacgccaactcaagtggcacgctgcatcgacagcctgggcatcggcttcatgttcgcgcaaagtcaccactcggccatgaaacatgccgctggcccacgtcgagaactggggttgcgcaccctgttcaatatgctcggcccgcttacgaatccggccggagtgaagcaccaggtggtcggtgtgttcgcgcaaaccctttgccgcccgctggctgaggtgctgcagcgcctggggagcaagcatgtgctggtcgtgcactcgaaggatggtctggacgagttcagcctggctgcacccaccttcgtcgccgaactgaaaaatgacgaaatcactgaatattgggtcgagccggaagacctcggcatgaagagtcagagccttcatggcctggctgtcgagagcccgcaggcttcgctggagttgatccgcgatgcgctgggccggcgcaagaccgagaacggtcagaaggccgccgagatgatcgtgcttaatgctggcgcggcactgtatgcagccgaccatgccatgagcctgaaagccggtgtagaactggcccatgatgtactgcacaccggcctggcctgggaaaagctgcaggaattgggtgcctttactgcagtattcaaggtggagaacgaagcatgagtgtgccgacggtgctggaaaggatcattgcccgcaagtttcaggaagtggccgagcgcagtgcgcacgtcagcctcgccgaactggagggcctggccaaggccgctgacgccccgcgaggcttcgccaacgcgctgatcgagcaggccaagcgcaagcagcccgcggtgattgccgaaatcaagaaagcttcgccaagcaagggcgtgatccgcgagcacttcgtgccagcggaaatcgcggtcagctacgagaagggcggggccacctgcctgtcggtgttgaccgatgtcgattatttccagggtgccgatgagtacttgcagcaggcccgcgcggcggtttcgctgccggtgatccgcaaggacttcatggtcgacccttaccagatcgtcgaagcccgggccctgggggcagattgcgtactgctgatcgtgtcggcgctggatgacgtgaagatggctgaactggccgccactgccaaggacgtcggcctcgacgtgctggtggaagtgcacgatggcgatgaactggagcgcgcgctgaaaaccctggatacgccgctggtgggggtgaacaaccgcaacctgcacaccttcgaggtcagcctggaaaccacccttgacctgctgccgcgcattccgcgtgaccgtctggcgattaccgaaagcggtattctcaaccgggccgatgtggagctgatggcaatcaacgaggtttactcgttcctggtgggtgaggcgttcatgcgcgccgagcagcctggcctggaattacagcggctgttcttccccgagcaggtgaagaagactgttcagcaactggactga

SEQ ID NO: 64 - DNA, 1104 bp, Corynebacterium glutamicum
atggctgacatgtccgaacaggagctcaaggcgctgcgcgtacgcatcgacagcctcgacgagaaaattctcgagctgatcagcgaccgcgcccgctgcgccgaagaagtggcccgggtcaagactgcctcgctgaaagaaggcgagaagccggtgttctaccgtcccgagcgtgaagctgcggtgctcaagcgcgtgatggaacgcaacaagggcccgctgggcaacgaagagatggcgcggctgttccgcgaaatcatgtcgtcgtgcctggccctggaagagccgctgaaaatcgcctacctcggccctgaaggtaccttcacccaggcggcggccatgaagcacttcggccacgcggtgatcagtcggccgatggcggccatcgacgaagtgttccgtgaagtggcggccggtgccgtcaacttcggtgtggtgccggtggaaaactccactgaaggtgcggtcagccacaccctggacagcttcctcgagcatgacatggtgatttgcggtgaggtcgagctgcgtatccaccaccacctgctggtgggcgagaacaccaagaccgacagcatcacccgcatctactcccacgcccagtcgctggcccagtgccgaaagtggctggacgctcactacccgaacgtggagcgcgtggccgtttcgagcaatgccgaagcggccaagcgggtcaagggtgagtggaactcggcggcgatcgccggcgatatggcggccaacctgtacggcctgacccgtctggccgagaagatcgaagaccgcccggacaactccacgcgcttcctgatgatcggtaaccaggaagtaccgccgaccggcgacgacaagacctcgatcatcgtttcgatgagcaacaagccaggtgcgttgcatgagttgctggtgccgttctatcagaacggcatcgacctgacccgcatcgagacccgcccgtcgcgcagcggcaagtggacctacgtgttcttcatcgacttcgtcggccaccaccgcgacccgctgatcaaggcggtgctcgagcagatcagccaggaggctgtggcgctgaaggtgctgggctcttatccgaaggcggtgctttga

SEQ ID NO: 65 - DNA, 8 bp, Artificial Sequence
  Artificial sequence
atggctga

SEQ ID NO: 66 - DNA, 21 bp, Artificial Sequence
  Artificial sequence
tatgccgtgttgaatgccatt

SEQ ID NO: 67 - DNA, 45 bp, Artificial Sequence
  Artificial sequence
cccgggatccactaaacttaaacacagtgttgctggagaagtcat

SEQ ID NO: 68 - DNA, 48 bp, Artificial Sequence
  Artificial sequence
tgtttaagtttagtggatcccggggaaaaggagtcttccaatgactag

SEQ ID NO: 69 - DNA, 21 bp, Artificial Sequence
  Artificial sequence
ccagatcgacgttttcctggc

SEQ ID NO: 70 - DNA, 50 bp, Artificial Sequence
  Artificial sequence
gccctgcaggtaaaaaaaggatttgattcatgacttctccagcaacactg

SEQ ID NO: 71 - DNA, 50 bp, Artificial Sequence
  Artificial sequence
gccctgcaggtaaaaaaaggatttgattcgtgacttctccagcaacactg

SEQ ID NO: 72 - DNA, 50 bp, Artificial Sequence
  Artificial sequence
gccctgcaggtaaaaaaaggatttgattcttgacttctccagcaacactg

SEQ ID NO: 73 - DNA, 44 bp, Artificial Sequence
  Artificial sequence
gccctgcaggtaaaaaaaggattatgacttctccagcaacactg

SEQ ID NO: 74 - DNA, 44 bp, Artificial Sequence; identical to SEQ ID NO: 73
  Artificial sequence

SEQ ID NO: 75 - DNA, 44 bp, Artificial Sequence
  Artificial Sequence, synthetic
gccctgcaggtaaaaaaaggattttgacttctccagcaacactg

SEQ ID NO: 76 - DNA, 31 bp, Artificial Sequence
  Artificial Sequence, synthetic
cccgggatccctagtcattggaagactcctt

SEQ ID NO: 77 - DNA, 45 bp, Artificial Sequence
  Artificial Sequence, synthetic
aatcctttttttacctgcagggcttagttcgcgagaagctgttcg

SEQ ID NO: 78 - DNA, 21 bp, Artificial Sequence
  Artificial Sequence, synthetic
aaggagtcttccaatgactag

SEQ ID NO: 79 - DNA, 21 bp, Artificial Sequence
  Artificial Sequence, synthetic
gtctccccaatcaaatcatca

SEQ ID NO: 80 - DNA, 42 bp, Artificial Sequence
  Artificial Sequence, synthetic
cccgggatccactaaacttaaacagtcacctgcattagtcat

SEQ ID NO: 81 - DNA, 42 bp, Artificial Sequence
  Artificial Sequence, synthetic
tgtttaagtttagtggatcccgggcgcggaaaactcggataa

SEQ ID NO: 82 - DNA, 21 bp, Artificial Sequence
  Artificial Sequence, synthetic
tgatgatgtgcccgtccacag

SEQ ID NO: 83 - DNA, 47 bp, Artificial Sequence
  Artificial Sequence, synthetic
gccctgcaggacgtggcagaatagtgtgcatgactaatgcaggtgac

SEQ ID NO: 84 - DNA, 47 bp, Artificial Sequence
  Artificial Sequence, synthetic
gccctgcaggacgtggcagaatagtgtgcgtgactaatgcaggtgac

SEQ ID NO: 85 - DNA, 47 bp, Artificial Sequence
  Artificial Sequence, synthetic
gccctgcaggacgtggcagaatagtgtgcttgactaatgcaggtgac

SEQ ID NO: 86 - DNA, 42 bp, Artificial Sequence
  Artificial Sequence, synthetic
gccctgcaggacgtggcagaatagatgactaatgcaggtgac

SEQ ID NO: 87 - DNA, 42 bp, Artificial Sequence
  Artificial Sequence, synthetic
gccctgcaggacgtggcagaataggtgactaatgcaggtgac

SEQ ID NO: 88 - DNA, 42 bp, Artificial Sequence
  Artificial Sequence, synthetic
gccctgcaggacgtggcagaatagttgactaatgcaggtgac

SEQ ID NO: 89 - DNA, 31 bp, Artificial Sequence
  Artificial Sequence, synthetic
cccgggatccttatccgagttttccgcgtcc

SEQ ID NO: 90 - DNA, 45 bp, Artificial Sequence; identical to SEQ ID NO: 77
  Artificial Sequence, synthetic

SEQ ID NO: 91 - DNA, 21 bp, Artificial Sequence
  Artificial Sequence, synthetic
aaggagtcttccaatgactag

SEQ ID NO: 92 - DNA, 11 bp, Artificial Sequence
  Artificial Sequence, synthetic
agccctgcagg

SEQ ID NO: 93 - DNA, 525 bp, Escherichia coli; identical to SEQ ID NO: 59

SEQ ID NO: 94 - DNA, 573 bp, Corynebacterium glutamicum; identical to SEQ ID NO: 60

SEQ ID NO: 95 - DNA, 1434 bp, Corynebacterium glutamicum
gtggcgtttgaaaccccggaagaaattgtcaagttcatcaaggatgaaaacgtcgagttcgttgacgttcgattcaccgaccttcccggcaccgagcagcacttcagcatcccagctgccagcttcgatgcagatacaatcgaagaaggtctcgcattcgacggatcctcgatccgtggcttcaccacgatcgacgaatctgacatgaatctcctgccagacctcggaacggccacccttgatccattccgcaaggcaaagaccctgaacgttaagttcttcgttcacgatcctttcacccgcgaggcattctcccgcgacccacgcaacgtggcacgcaaggcagagcagtacctggcatccaccggcattgcagacacctgcaacttcggcgccgaggctgagttctacctcttcgactccgttcgctactccaccgagatgaactccggcttctacgaagtagataccgaagaaggctggtggaaccgtggcaaggaaaccaacctcgacggcaccccaaacctgggcgcaaagaaccgcgtcaagggtggctacttcccagtagcaccatacgaccaaaccgttgacgtgcgcgatgacatggttcgcaacctcgcagcttccggcttcgctcttgagcgtttccaccacgaagtcggtggcggacagcaggaaatcaactaccgcttcaacaccatgctccacgcggcagatgatatccagaccttcaagtacatcatcaagaacaccgctcgcctccacggcaaggctgcaaccttcatgcctaagccactggctggcgacaacggttccggcatgcacgctcaccagtccctctggaaggacggcaagccactcttccacgatgagtccggctacgcaggcctgtccgacatcgcccgctactacatcggcggcatcctgcaccacgcaggcgctgttctggcgttcaccaacgcaaccctgaactcctaccaccgtctggttccaggcttcgaggctccaatcaacctggtgtactcacagcgcaaccgttccgctgctgtccgtatcccaatcaccggatccaacccgaaggcaaagcgcatcgaattccgcgctccagacccatcaggcaacccatacctgggctttgcagcgatgatgatggccggcctcgacggcatcaagaaccgcatcgagccacacgctccagtggacaaggacctctacgaactaccaccagaggaagctgcatccattccacaggcaccaacctccctggaagcatccctgaaggcactgcaggaagacaccgacttcctcaccgagtctgacgtcttcaccgaggatctcatcgaggcgtacatccagtacaagtacgacaacgagatctccccagttcgcctgcgcccaaccccgcaggaattcgaattgtacttcgactgctaa

SEQ ID NO: 96 - DNA, 1857 bp, Corynebacterium glutamicum
atgcgtacatccattgccactgtttgtttgtccggaactcttgctgaaaagctgcgcgcagctgcagatgctggatttgatggtgtggaaatcttcgagcaggacttggtggtttccccgcattcggcagagcagattcgtcagcgggctcaggatttgggattaaccctggatctgttccagccgtttcgagatttcgaaggtgtggaagaagagcagtttctgaagaatctgcaccgcttggaagagaagttcaagctgatgaacaggcttggcattgagatgatcttgttgtgttccaatgtgggcaccgcgaccatcaatgatgatgaccttttcgtggagcagttgcatcgtgcagcagatttggctgagaagtacaacgtcaagattgcttatgaagcgttggcgtggggcaagtttgtcaatgattttgagcatgcgcatgcacttgtggagaaggtgaatcacaaggcgctgggaacctgcttggatacgttccatattctttcccgtggttgggaaaccgacgaggtggaaaacatcccggcggagaagattttctttgttcagttggcggatgcaccgaagctgagcatggacattttgtcctggtcgcgtcaccaccgtgttttccctggtgaaggcgatttcgatctggtgaaattcatggttcatctggccaagacgggttatgatggcccgatttctttggaaatcttcaacgattccttccgcaaggccgaggttggtcgcaccgcgattgatgggttgcgttctttgcgttggttggaagatcagacctggcatgcgctaaatgctgaggatcgtccaagcgcactagagctgcgtgcacttcctgaggtcgcggaacctgaaggcgttgatttcattgagatcgccactggacgtttgggtgagaccattcgggttcttcatcaattgggtttccgcttgggtggtcatcactgcagtaagcaggattaccaggtatggacccagggcgatgtgcgcattgtggtgtgtgatcgtggggccaccggggctccaaccacgatctctgcgatgggctttgacacccctgatccagaagccgcgcatgcccgtgcggaattgctgcgggctcagacaattgatcgtccccacatcgagggtgaagttgaccttaaaggtgtgtacgcgccggatggggtggagctgtttttcgcggggccgagccccgatggaatgcccgagtggctgccggagttcggcgtcgaaaagcaagaagctggtctcattgaagccatcgaccacgtcaatttcgcccagccgtggcaacattttgatgaggcagtgctgttttacaccgcgctgatggcgttagagactgtgcgtgaggatgagttcccgagcccaattggtttggtgcgcaatcaggtgatgcgttcgccgaatgatgcggtgcggttgctgctcagcgtggcgccggaggacggtgagcagggagatttcctcaacgcggcctacccggagcacattgcgttggccacggcggacatcgtggcggtggctgaacgtgcgcgcaaacgaggcctggatttcttgcccgtcccagagaattactacgacgatgtgcaggcgcgttttgatttgccgcaggagttcttggacacactcaaggaaaaccacctgctttacgactgcgacgagaacggcgagttcctccacttttacacccgcacgttgggcacgctgttcttcgaagtggtggaacgccgcggcggttttgcaggttggggcgaaacaaacgctccggtgcggttagcggcgcagtatcgtgaggtgcgggacctcgagcggggaatccccaactag

SEQ ID NO: 97 - DNA, 39 bp, Artificial Sequence
  Primer
ttagaggagacaccatatggcgtttgaaaccccggaaga

SEQ ID NO: 98 - DNA, 42 bp, Artificial Sequence
  Primer Ex-glnA-2
gaaccatgggctagcctcgagttagcagtcgaagtacaattc

SEQ ID NO: 99 - DNA, 50 bp, Artificial Sequence
  Primer Ex-aroL-1
ggccctgcagggaaaggaggcccttcagatgacacaacctctttttctga

SEQ ID NO: 100 - DNA, 31 bp, Artificial Sequence
  Primer Ex-aroL-2
cccgggatcctcaacaattgatcgtctgtgc

SEQ ID NO: 101 - DNA, 50 bp, Artificial Sequence
  Primer Ex-aroK-1
ggccctgcagggaaaggaggcccttcagatgaatgatcaaattcacttag

SEQ ID NO: 102 - DNA, 32 bp, Artificial Sequence
  Primer Ex-aroK-2
cccgggatccttaatcgatttctagatgatgc

SEQ ID NO: 103 - DNA, 45 bp, Artificial Sequence
  Primer JK038f
attcgagctcggtacccggggatccactacatcgaaaccggcatc

SEQ ID NO: 104 - DNA, 29 bp, Artificial Sequence
  Primer JK039r
ctgaactcgagtcagccatgctccttctc

SEQ ID NO: 105 - DNA, 34 bp, Artificial Sequence
  Primer JK040f
gcatggctgactcgagttcaggggccttggggct

SEQ ID NO: 106 - DNA, 44 bp, Artificial Sequence
  Primer JK041r
tagaagcttgcatgcctgcaggcagtgagtcgaccaggccaaag

SEQ ID NO: 107 - DNA, 21 bp, Artificial Sequence
  Primer Ko-csm-1
cttgccgacgagcgtagaaat

SEQ ID NO: 108 - DNA, 21 bp, Artificial Sequence
  Primer Ko-csm-2
gttgaggactaccttgacttg

SEQ ID NO: 109 - DNA, 54 bp, Artificial Sequence
  Primer Ex-aroG-1
gccctgcaggagatctgaaaggaggcccttcagatgaattatcagaacgacgat

SEQ ID NO: 110 - DNA, 31 bp, Artificial Sequence
  Primer Ex-aroG-2
cccgggatccttacccgcgacgcgcttttac